European Patent Application EP 4 137 509 A1, published February 22, 2023. Title: COMBINATIONS OF MRNAS ENCODING IMMUNE MODULATING POLYPEPTIDES AND USES THEREOF. Applicant: MODERNATX, INC. Application EP 17727999.9. The sequence listing filed with the application follows.

SEQUENCE LISTING (198 sequences)

SEQ ID NO: 1 - protein, 328 aa, Homo sapiens
  Amino acid sequence of human IL-23 IL-12p40 subunit (Precursor)
MCHQQLVISWFSLVFLASPLVAIWELKKDVYVVELDWYPDAPGEMVVLTCDTPEEDGITWTLDQSSEVLGSGKTLTIQVKEFGDAGQYTCHKGGEVLSHSLLLLHKKEDGIWSTDILKDQKEPKNKTFLRCEAKNYSGRFTCWWLTTISTDLTFSVKSSRGSSDPQGVTCGAATLSAERVRGDNKEYEYSVECQEDSACPAAEESLPIEVMVDAVHKLKYENYTSSFFIRDIIKPDPPKNLQLKPLKNSRQVEVSWEYPDTWSTPHSYFSLTFCVQVQGKSKREKKDRVFTDKTSATVICRKNASISVRAQDRYYSSSWSEWASVPCS

SEQ ID NO: 2 - protein, 133 aa, Homo sapiens
  TNFSF4 isoform 2
MVSHRYPRIQSIKVQFTEYKKEKGFILTSQKEDEIMKVQNNSVIINCDGFYLISLKGYFSQEVNISLHYQKDEEPLFQLKKVRSVNSLMVASLTYKDKVYLNVTTDNTSLDDFHVNGGELILIHQNPGEFCVL

SEQ ID NO: 3 - protein, 306 aa, Homo sapiens
  Amino acid sequence of human IL-23 IL-12p40 subunit (Mature)
IWELKKDVYVVELDWYPDAPGEMVVLTCDTPEEDGITWTLDQSSEVLGSGKTLTIQVKEFGDAGQYTCHKGGEVLSHSLLLLHKKEDGIWSTDILKDQKEPKNKTFLRCEAKNYSGRFTCWWLTTISTDLTFSVKSSRGSSDPQGVTCGAATLSAERVRGDNKEYEYSVECQEDSACPAAEESLPIEVMVDAVHKLKYENYTSSFFIRDIIKPDPPKNLQLKPLKNSRQVEVSWEYPDTWSTPHSYFSLTFCVQVQGKSKREKKDRVFTDKTSATVICRKNASISVRAQDRYYSSSWSEWASVPCS

SEQ ID NO: 4 - protein, 189 aa, Homo sapiens
  Amino acid sequence of human IL-23 IL-23p19 subunit (Precursor)
MLGSRAVMLLLLLPWTAQGRAVPGGSSPAWTQCQQLSQKLCTLAWSAHPLVGHMDLREEGDEETTNDVPHIQCGDGCDPQGLRDNSQFCLQRIHQGLIFYEKLLGSDIFTGEPSLLPDSPVGQLHASLLGLSQLLQPEGHHWETQQIPSLSPSQPWQRLLLRFKILRSLQAFVAVAARVFAHGAATLSP

SEQ ID NO: 5 - protein, 170 aa, Homo sapiens
  Amino acid sequence of human IL-23 IL-23p19 subunit (Mature)
RAVPGGSSPAWTQCQQLSQKLCTLAWSAHPLVGHMDLREEGDEETTNDVPHIQCGDGCDPQGLRDNSQFCLQRIHQGLIFYEKLLGSDIFTGEPSLLPDSPVGQLHASLLGLSQLLQPEGHHWETQQIPSLSPSQPWQRLLLRFKILRSLQAFVAVAARVFAHGAATLSP

SEQ ID NO: 6 - DNA, 986 bp, Homo sapiens
  Nucleotide sequence of human IL-23 IL-12p40 subunit (Precursor)
atgtgtcaccagcagttggtcatctcttggttttccctggtttttctggcatctcccctcgtggccatatgggaactgaagaaagatgtttatgtcgtagaattggattggtatccggatgcccctggagaaatggtggtcctcacctgtgacacccctgaagaagatggtatcacctggaccttggaccagagcagtgaggtcttaggctctggcaaaaccctgaccatccaagtcaaagagtttggagatgctggccagtacacctgtcacaaaggaggcgaggttctaagccattcgctcctgctgcttcacaaaaaggaagatggaatttggtccactgatattttaaaggaccagaaagaacccaaaaataagacctttctaagatgcgaggccaagaattattctggacgtttcacctgctggtggctgacgacaatcagtactgatttgacattcagtgtcaaaagcagcagaggctcttctgacccccaaggggtgacgtgcggagctgctacactctctgcagagagagtcagaggggacaacaaggagtatgagtactcagtggagtgccaggaggacagtgcctgcccagctgctgaggagagtctgcccattgaggtcatggtggatgccgttcacaagctcaagtatgaaaactacaccagcagcttcttcatcagggacatcatcaaacctgacccacccaagaacttgcagctgaagccattaaagaattctcggcaggtggaggtcagctgggagtaccctgacacctggagtactccacattcctacttctccctgacattctgcgttcaggtccagggcaagagcaagagagaaaagaaagatagagtcttcacggacaagacctcagccacggtcatctgccgcaaaaatgccagcattagcgtgcgggcccaggaccgctactatagctcatcttggagcgaatgggcatctgtgccctgcagtta

SEQ ID NO: 7 - DNA, 920 bp, Homo sapiens
  Nucleotide sequence of human IL-23 IL-12p40 subunit (Mature)
atatgggaactgaagaaagatgtttatgtcgtagaattggattggtatccggatgcccctggagaaatggtggtcctcacctgtgacacccctgaagaagatggtatcacctggaccttggaccagagcagtgaggtcttaggctctggcaaaaccctgaccatccaagtcaaagagtttggagatgctggccagtacacctgtcacaaaggaggcgaggttctaagccattcgctcctgctgcttcacaaaaaggaagatggaatttggtccactgatattttaaaggaccagaaagaacccaaaaataagacctttctaagatgcgaggccaagaattattctggacgtttcacctgctggtggctgacgacaatcagtactgatttgacattcagtgtcaaaagcagcagaggctcttctgacccccaaggggtgacgtgcggagctgctacactctctgcagagagagtcagaggggacaacaaggagtatgagtactcagtggagtgccaggaggacagtgcctgcccagctgctgaggagagtctgcccattgaggtcatggtggatgccgttcacaagctcaagtatgaaaactacaccagcagcttcttcatcagggacatcatcaaacctgacccacccaagaacttgcagctgaagccattaaagaattctcggcaggtggaggtcagctgggagtaccctgacacctggagtactccacattcctacttctccctgacattctgcgttcaggtccagggcaagagcaagagagaaaagaaagatagagtcttcacggacaagacctcagccacggtcatctgccgcaaaaatgccagcattagcgtgcgggcccaggaccgctactatagctcatcttggagcgaatgggcatctgtgccctgcagtta

SEQ ID NO: 8 - DNA, 567 bp, Homo sapiens
  Nucleotide sequence of human IL-23 IL-23p19 subunit (Precursor)
atgctggggagcagagctgtaatgctgctgttgctgctgccctggacagctcagggcagagctgtgcctgggggcagcagccctgcctggactcagtgccagcagctttcacagaagctctgcacactggcctggagtgcacatccactagtgggacacatggatctaagagaagagggagatgaagagactacaaatgatgttccccatatccagtgtggagatggctgtgacccccaaggactcagggacaacagtcagttctgcttgcaaaggatccaccagggtctgattttttatgagaagctgctaggatcggatattttcacaggggagccttctctgctccctgatagccctgtggcgcagcttcatgcctccctactgggcctcagccaactcctgcagcctgagggtcaccactgggagactcagcagattccaagcctcagtcccagccagccatggcagcgtctccttctccgcttcaaaatccttcgcagcctccaggcctttgtggctgtagccgcccgggtctttgcccatggagcagcaaccctgagtccc

SEQ ID NO: 9 - DNA, 510 bp, Homo sapiens
  Nucleotide sequence of human IL-23 IL-23p19 subunit (Mature)
agagctgtgcctgggggcagcagccctgcctggactcagtgccagcagctttcacagaagctctgcacactggcctggagtgcacatccactagtgggacacatggatctaagagaagagggagatgaagagactacaaatgatgttccccatatccagtgtggagatggctgtgacccccaaggactcagggacaacagtcagttctgcttgcaaaggatccaccagggtctgattttttatgagaagctgctaggatcggatattttcacaggggagccttctctgctccctgatagccctgtggcgcagcttcatgcctccctactgggcctcagccaactcctgcagcctgagggtcaccactgggagactcagcagattccaagcctcagtcccagccagccatggcagcgtctccttctccgcttcaaaatccttcgcagcctccaggcctttgtggctgtagccgcccgggtctttgcccatggagcagcaaccctgagtccc

SEQ ID NO: 10 - protein, 169 aa, Homo sapiens
  Amino acid sequence of IL-36-gamma (Precursor)
MRGTPGDADGGGRAVYQSMCKPITGTINDLNQQVWTLQGQNLVAVPRSDSVTPVTVAVITCKYPEALEQGRGDPIYLGIQNPEMCLYCEKVGEQPTLQLKEQKIMDLYGQPEPVKPFLFYRAKTGRTSTLESVAFPDWFIASSKRDQPIILTSELGKSYNTAFELNIND

SEQ ID NO: 11 - DNA, 507 bp, Homo sapiens
  Nucleotide sequence of IL-36-gamma (Precursor)
atgagaggcactccaggagacgctgatggtggaggaagggccgtctatcaatcaatgtgtaaacctattactgggactattaatgatttgaatcagcaagtgtggacccttcagggtcagaaccttgtggcagttccacgaagtgacagtgtgaccccagtcactgttgctgttatcacatgcaagtatccagaggctcttgagcaaggcagaggggatcccatttatttgggaatccagaatccagaaatgtgtttgtattgtgagaaggttggagaacagcccacattgcagctaaaagagcagaagatcatggatctgtatggccaacccgagcccgtgaaacccttccttttctaccgtgccaagactggtaggacctccacccttgagtctgtggccttcccggactggttcattgcctcctccaagagagaccagcccatcattctgacttcagaacttgggaagtcatacaacactgcctttgaattaaatataaatgac

SEQ ID NO: 12 - protein, 152 aa, Homo sapiens
  Amino acid sequence of IL-36-gamma (Mature)
SMCKPITGTINDLNQQVWTLQGQNLVAVPRSDSVTPVTVAVITCKYPEALEQGRGDPIYLGIQNPEMCLYCEKVGEQPTLQLKEQKIMDLYGQPEPVKPFLFYRAKTGRTSTLESVAFPDWFIASSKRDQPIILTSELGKSYNTAFELNIND

SEQ ID NO: 13 - DNA, 456 bp, Homo sapiens
  Nucleotide sequence of IL-36-gamma (Mature) (CCDS2108.1, nt 52-507)
tcaatgtgtaaacctattactgggactattaatgatttgaatcagcaagtgtggacccttcagggtcagaaccttgtggcagttccacgaagtgacagtgtgaccccagtcactgttgctgttatcacatgcaagtatccagaggctcttgagcaaggcagaggggatcccatttatttgggaatccagaatccagaaatgtgtttgtattgtgagaaggttggagaacagcccacattgcagctaaaagagcagaagatcatggatctgtatggccaacccgagcccgtgaaacccttccttttctaccgtgccaagactggtaggacctccacccttgagtctgtggccttcccggactggttcattgcctcctccaagagagaccagcccatcattctgacttcagaacttgggaagtcatacaacactgcctttgaattaaatataaatgac

SEQ ID NO: 14 - protein, 20 aa, Homo sapiens
  Amino acid sequence of IgKV4 signal peptide
MVLQTQVFISLLLWISGAYG

SEQ ID NO: 15 - DNA, 60 bp, Homo sapiens
  Nucleotide sequence of IgKV4 signal peptide (IMGT Z00023, nt 1-60)
atggtgttgcagacccaggtcttcatttctctgttgctctggatctctggtgcctacggg

SEQ ID NO: 16 - protein, 172 aa, Artificial Sequence
  Synthetic: hIGKV4-hIL-36g construct (protein)
MVLQTQVFISLLLWISGAYGSMCKPITGTINDLNQQVWTLQGQNLVAVPRSDSVTPVTVAVITCKYPEALEQGRGDPIYLGIQNPEMCLYCEKVGEQPTLQLKEQKIMDLYGQPEPVKPFLFYRAKTGRTSTLESVAFPDWFIASSKRDQPIILTSELGKSYNTAFELNIND

SEQ ID NO: 17 - DNA, 516 bp, Artificial Sequence
  Synthetic: hIGKV4-hIL-36g construct (RNA)
atggtgttgcagacccaggtcttcatttctctgttgctctggatctctggtgcctacgggtcaatgtgtaaacctattactgggactattaatgatttgaatcagcaagtgtggacccttcagggtcagaaccttgtggcagttccacgaagtgacagtgtgaccccagtcactgttgctgttatcacatgcaagtatccagaggctcttgagcaaggcagaggggatcccatttatttgggaatccagaatccagaaatgtgtttgtattgtgagaaggttggagaacagcccacattgcagctaaaagagcagaagatcatggatctgtatggccaacccgagcccgtgaaacccttccttttctaccgtgccaagactggtaggacctccacccttgagtctgtggccttcccggactggttcattgcctcctccaagagagaccagcccatcattctgacttcagaacttgggaagtcatacaacactgcctttgaattaaatataaatgac

SEQ ID NO: 18 - DNA, 1515 bp, Artificial Sequence
  Synthetic: Codon optimized human IL-23 sequence
atgtgtcaccagcagttggtcatctcttggttttccctggtatttctggcatctcccctcgtggccatatgggaactgaagaaagatgtttatgtcgtagaattggattggtatccggatgcccctggagaaatggtggtcctcacctgtgacacccctgaagaagatggtatcacctggaccttggaccagagcagtgaggtcttaggctctggcaagaccctgaccatccaagtcaaagagtttggagatgctggccagtacacctgtcacaaaggaggcgaggttctaagccattcgctcctgctgcttcacaagaaggaagatggaatttggtccactgatattttaaaggaccagaaagaacccaagaataagacctttctaagatgcgaggccaagaattattctggacgtttcacctgctggtggctgacgacaatcagtactgatttgacattcagtgtcaagagcagcagaggctcttctgacccgcaaggggtgacgtgcggagctgctacactctctgcagagagagtcagaggggacaacaaggagtatgagtactcagtggagtgccaggaggacagtgcctgcccagctgctgaggagagtctgcccattgaggtcatggtggatgccgttcacaagctcaagtatgagaactacaccagcagcttcttcatcagggacatcatcaaacctgacccacccaagaacttgcagctgaagccattaaagaattctcggcaggtggaggtcagctgggagtaccctgacacctggagtactccacattcctacttctccctgacattctgcgttcaggtccagggcaagagcaagagagagaagaaagatagagtcttcacggacaagacctcagccacggtcatctgccgcaagaatgccagcattagcgtgcgggcccaggaccgctactatagctcatcttggagcgaatgggcatctgtgccctgcagtggcggaggtggcggagggagcagagctgtgcctggcggcagcagccctgcctggactcagtgccagcagctttcacagaagctctgcacactggcctggagtgcacatccactagtgggacacatggatctaagagaagagggagatgaagagactacaaatgatgttccccatatccagtgtggagatggctgtgacccgcaaggactcagggacaacagtcagttctgcttgcaaaggatccaccagggtctgatcttttatgagaagctgctaggatcggatattttcacaggggagccttctctgctccctgatagccctgtgggccagcttcatgcctccctactgggcctcagccaactcctgcagcctgagggtcaccactgggagactcagcagattccaagcctcagtcccagccagccatggcagcgtctccttctccgcttcaagatccttcgcagcctccaggcctttgtggctgtagccgcccgggtctttgcccatggagcagcaaccctgagtccc

SEQ ID NO: 19 - DNA, 1515 bp, Artificial Sequence
  Synthetic: Codon optimized human IL-23 sequence
atgtgtcaccagcagttggtcatctcttggttttccctggtatttctggcatctcccctcgtggccatatgggaactgaagaaagatgtttatgtcgtagaattggattggtatccggatgcccctggagaaatggtggtcctcacctgtgacacccctgaagaagatggtatcacctggaccttggaccagagcagtgaggtcttaggctctggcaagaccctgaccatccaagtcaaagagtttggagatgctggccagtacacctgtcacaaaggaggcgaggttctaagccattcgctcctgctgcttcacaagaaggaagatggaatttggtccactgatattttaaaggaccagaaagaacccaagaataagacctttctaagatgcgaggccaagaattattctggacgtttcacctgctggtggctgacgacaatcagtactgatttgacattcagtgtcaagagcagcagaggctcttctgacccccaaggggtgacgtgcggagctgctacactctctgcagagagagtcagaggggacaacaaggagtatgagtactcagtggagtgccaggaggacagtgcctgcccagctgctgaggagagtctgcccattgaggtcatggtggatgccgttcacaagctcaagtatgagaactacaccagcagcttcttcatcagggacatcatcaaacctgacccacccaagaacttgcagctgaagccattaaagaattctcggcaggtggaggtcagctgggagtaccctgacacctggagtactccacattcctacttctccctgacattctgcgttcaggtccagggcaagagcaagagagagaagaaagatagagtcttcacggacaagacctcagccacggtcatctgccgcaagaatgccagcattagcgtgcgggcccaggaccgctactatagctcatcttggagcgaatgggcatctgtgccctgcagtggcggagggggcggagggagcagagctgtgcctgggggcagcagccctgcctggactcagtgccagcagctttcacagaagctctgcacactggcctggagtgcacatccactagtgggacacatggatctaagagaagagggagatgaagagactacaaatgatgttccccatatccagtgtggagatggctgtgacccccaaggactcagggacaacagtcagttctgcttgcaaaggatccaccagggtctgatcttttatgagaagctgctaggatcggatattttcacaggggagccttctctgctccctgatagccctgtgggccagcttcatgcctccctactgggcctcagccaactcctgcagcctgagggtcaccactgggagactcagcagattccaagcctcagtcccagccagccatggcagcgtctccttctccgcttcaagatccttcgcagcctccaggcctttgtggctgtagccgcccgggtctttgcccatggagcagcaaccctgagtccc

SEQ ID NO: 20 - DNA, 1515 bp, Artificial Sequence
  Synthetic: Codon optimized human IL-23 sequence
atgtgtcaccagcagttggtcatctcttggttttccctggtttttctggcatctcccctcgtggccatatgggaactgaagaaagatgtttatgtcgtagaattggattggtatccggatgcccctggagaaatggtggtcctcacctgtgacacccctgaagaagatggtatcacctggaccttggaccagagcagtgaggtcttaggctctggcaaaaccctgaccatccaagtcaaagagtttggagatgctggccagtacacctgtcacaaaggaggcgaggttctaagccattcgctcctgctgcttcacaaaaaggaagatggaatttggtccactgatattttaaaggaccagaaagaacccaaaaataagacctttctaagatgcgaggccaagaattattctggacgtttcacctgctggtggctgacgacaatcagtactgatttgacattcagtgtcaaaagcagcagaggctcttctgacccccaaggggtgacgtgcggagctgctacactctctgcagagagagtcagaggggacaacaaggagtatgagtactcagtggagtgccaggaggacagtgcctgcccagctgctgaggagagtctgcccattgaggtcatggtggatgccgttcacaagctcaagtatgaaaactacaccagcagcttcttcatcagggacatcatcaaacctgacccacccaagaacttgcagctgaagccattaaagaattctcggcaggtggaggtcagctgggagtaccctgacacctggagtactccacattcctacttctccctgacattctgcgttcaggtccagggcaagagcaagagagaaaagaaagatagagtcttcacggacaagacctcagccacggtcatctgccgcaaaaatgccagcattagcgtgcgggcccaggaccgctactatagctcatcttggagcgaatgggcatctgtgccctgcagtggcggagggggcggagggagcagagctgtgcctgggggcagcagccctgcctggactcagtgccagcagctttcacagaagctctgcacactggcctggagtgcacatccactagtgggacacatggatctaagagaagagggagatgaagagactacaaatgatgttccccatatccagtgtggagatggctgtgacccccaaggactcagggacaacagtcagttctgcttgcaaaggatccaccagggtctgattttttatgagaagctgctaggatcggatattttcacaggggagccttctctgctccctgatagccctgtgggccagcttcatgcctccctactgggcctcagccaactcctgcagcctgagggtcaccactgggagactcagcagattccaagcctcagtcccagccagccatggcagcgtctccttctccgcttcaaaatccttcgcagcctccaggcctttgtggctgtagccgcccgggtctttgcccatggagcagcaaccctgagtccc

SEQ ID NO: 21 - protein, 183 aa, Homo sapiens
  Tumor necrosis factor ligand superfamily member 4 isoform 1
MERVQPLEENVGNAARPRFERNKLLLVASVIQGLGLLLCFTYICLHFSALQVSHRYPRIQSIKVQFTEYKKEKGFILTSQKEDEIMKVQNNSVIINCDGFYLISLKGYFSQEVNISLHYQKDEEPLFQLKKVRSVNSLMVASLTYKDKVYLNVTTDNTSLDDFHVNGGELILIHQNPGEFCVL

SEQ ID NO: 22 - RNA, 85 nt, Artificial Sequence
  Synthetic: miR-122
ccuuagcagagcuguggagugugacaaugguguuugugucuaaacuaucaaacgccauuaucacacuaaauagcuacugcuaggc

SEQ ID NO: 23 - RNA, 22 nt, Artificial Sequence
  Synthetic: miR-122-3p
aacgccauuaucacacuaaaua

SEQ ID NO: 24 - RNA, 22 nt, Artificial Sequence
  Synthetic: miR-122-3p binding site
uauuuagugugauaauggcguu

SEQ ID NO: 25 - RNA, 22 nt, Artificial Sequence
  Synthetic: miR-122-5p
uggagugugacaaugguguuug

SEQ ID NO: 26 - RNA, 22 nt, Artificial Sequence
  Synthetic: miR-122-5p binding site
caaacaccauugucacacucca

SEQ ID NO: 27 - RNA, 47 nt, Artificial Sequence
  Synthetic: 5UTR-001
gggaaauaagagagaaaagaagaguaagaagaaauauaagagccacc

SEQ ID NO: 28 - RNA, 47 nt, Artificial Sequence
  Synthetic: 5UTR-002
gggagaucagagagaaaagaagaguaagaagaaauauaagagccacc

SEQ ID NO: 29 - RNA, 145 nt, Artificial Sequence
  Synthetic: 5UTR-003
ggaauaaaagucucaacacaacauauacaaaacaaacgaaucucaagcaaucaagcauucuacuucuauugcagcaauuuaaaucauuucuuuuaaagcaaaagcaauuuucugaaaauuuucaccauuuacgaacgauagcaac

SEQ ID NO: 30 - RNA, 42 nt, Artificial Sequence
  Synthetic: 5UTR-004
gggagacaagcuuggcauuccgguacuguugguaaagccacc

SEQ ID NO: 31 - RNA, 47 nt, Artificial Sequence; identical to SEQ ID NO: 28
  Synthetic: 5UTR-005

SEQ ID NO: 32 - RNA, 145 nt, Artificial Sequence; identical to SEQ ID NO: 29
  Synthetic: 5UTR-006

SEQ ID NO: 33 - RNA, 42 nt, Artificial Sequence; identical to SEQ ID NO: 30
  Synthetic: 5UTR-007

SEQ ID NO: 34 - RNA, 47 nt, Artificial Sequence
  Synthetic: 5UTR-008
gggaauuaacagagaaaagaagaguaagaagaaauauaagagccacc

SEQ ID NO: 35 - RNA, 47 nt, Artificial Sequence
  Synthetic: 5UTR-009
gggaaauuagacagaaaagaagaguaagaagaaauauaagagccacc

SEQ ID NO: 36 - RNA, 47 nt, Artificial Sequence
  Synthetic: 5UTR-010
gggaaauaagagaguaaagaacaguaagaagaaauauaagagccacc

SEQ ID NO: 37 - RNA, 47 nt, Artificial Sequence
  Synthetic: 5UTR-011
gggaaaaaagagagaaaagaagacuaagaagaaauauaagagccacc

SEQ ID NO: 38 - RNA, 47 nt, Artificial Sequence
  Synthetic: 5UTR-012
gggaaauaagagagaaaagaagaguaagaagauauauaagagccacc

SEQ ID NO: 39 - RNA, 47 nt, Artificial Sequence
  Synthetic: 5UTR-013
gggaaauaagagacaaaacaagaguaagaagaaauauaagagccacc

SEQ ID NO: 40 - RNA, 47 nt, Artificial Sequence
  Synthetic: 5UTR-014
gggaaauuagagaguaaagaacaguaaguagaauuaaaagagccacc

SEQ ID NO: 41 - RNA, 47 nt, Artificial Sequence
  Synthetic: 5UTR-015
gggaaauaagagagaauagaagaguaagaagaaauauaagagccacc

SEQ ID NO: 42 - RNA, 47 nt, Artificial Sequence
  Synthetic: 5UTR-016
gggaaauaagagagaaaagaagaguaagaagaaaauuaagagccacc

SEQ ID NO: 43 - RNA, 47 nt, Artificial Sequence
  Synthetic: 5UTR-017
gggaaauaagagagaaaagaagaguaagaagaaauuuaagagccacc

SEQ ID NO: 44 - RNA, 47 nt, Artificial Sequence; identical to SEQ ID NO: 27
  Synthetic: 5UTR-018

SEQ ID NO: 45 - RNA, 371 nt, Artificial Sequence
  Synthetic: 3UTR-001
gcgccugcccaccugccaccgacugcuggaacccagccagugggagggccuggcccaccagaguccugcucccucacuccucgccccgcccccugucccagagucccaccugggggcucucuccacccuucucagaguuccaguuucaaccagaguuccaaccaaugggcuccauccucuggauucuggccaaugaaauaucucccuggcaggguccucuucuuuucccagagcuccaccccaaccaggagcucuaguuaauggagagcucccagcacacucggagcuugugcuuugucuccacgcaaagcgauaaauaaaagcauugguggccuuuggucuuugaauaaagccugaguaggaagucuaga

SEQ ID NO: 46 - RNA, 568 nt, Artificial Sequence
  Synthetic: 3UTR-002
gccccugccgcucccacccccacccaucugggccccggguucaagagagagcggggucugaucucguguagccauauagaguuugcuucugagugucugcuuuguuuaguagaggugggcaggaggagcugaggggcuggggcugggguguugaaguuggcuuugcaugcccagcgaugcgccucccugugggaugucaucacccugggaaccgggaguggcccuuggcucacuguguucugcaugguuuggaucugaauuaauuguccuuucuucuaaaucccaaccgaacuucuuccaaccuccaaacuggcuguaaccccaaauccaagccauuaacuacaccugacaguagcaauugucugauuaaucacuggccccuugaagacagcagaaugucccuuugcaaugaggaggagaucugggcugggcgggccagcuggggaagcauuugacuaucuggaacuugugugugccuccucagguauggcagugacucaccugguuuuaauaaaacaaccugcaacaucucauggucuuugaauaaagccugaguaggaagucuaga

SEQ ID NO: 47 - RNA, 289 nt, Artificial Sequence
  Synthetic: 3UTR-003
acacacuccaccuccagcacgcgacuucucaggacgacgaaucuucucaaugggggggcggcugagcuccagccaccccgcagucacuuucuuuguaacaacuuccguugcugccaucguaaacugacacaguguuuauaacguguacauacauuaacuuauuaccucauuuuguuauuuuucgaaacaaagcccuguggaagaaaauggaaaacuugaagaagcauuaaagucauucuguuaagcugcguaaauggucuuugaauaaagccugaguaggaagucuaga

SEQ ID NO: 48 - RNA, 379 nt, Artificial Sequence
  Synthetic: 3UTR-004
caucacauuuaaaagcaucucagccuaccaugagaauaagagaaagaaaaugaagaucaaaagcuuauucaucuguuuuucuuuuucguugguguaaagccaacacccugucuaaaaaacauaaauuucuuuaaucauuuugccucuuuucucugugcuucaauuaauaaaaaauggaaagaaucuaauagagugguacagcacuguuauuuuucaaagauguguugcuauccugaaaauucuguagguucuguggaaguuccaguguucucucuuauuccacuucgguagaggauuucuaguuucuugugggcuaauuaaauaaaucauuaauacucuucuaauggucuuugaauaaagccugaguaggaagucuaga

SEQ ID NO: 49 - RNA, 118 nt, Artificial Sequence
  Synthetic: 3UTR-005
gcugccuucugcggggcuugccuucuggccaugcccuucuucucucccuugcaccuguaccucuuggucuuugaauaaagccugaguaggaaggcggccgcucgagcaugcaucuaga

SEQ ID NO: 50 - RNA, 908 nt, Artificial Sequence
  Synthetic: 3UTR-006
gccaagcccuccccaucccauguauuuaucucuauuuaauauuuaugucuauuuaagccucauauuuaaagacagggaagagcagaacggagccccaggccucuguguccuucccugcauuucugaguuucauucuccugccuguagcagugagaaaaagcuccuguccucccauccccuggacugggagguagauagguaaauaccaaguauuuauuacuaugacugcuccccagcccuggcucugcaaugggcacugggaugagccgcugugagccccugguccugaggguccccaccugggacccuugagaguaucaggucucccacgugggagacaagaaaucccuguuuaauauuuaaacagcaguguuccccaucuggguccuugcaccccucacucuggccucagccgacugcacagcggccccugcauccccuuggcugugaggccccuggacaagcagagguggccagagcugggaggcauggcccuggggucccacgaauuugcuggggaaucucguuuuucuucuuaagacuuuugggacaugguuugacucccgaacaucaccgacgcgucuccuguuuuucuggguggccucgggacaccugcccugcccccacgagggucaggacugugacucuuuuuagggccaggcaggugccuggacauuugccuugcuggacggggacuggggaugugggagggagcagacaggaggaaucaugucaggccugugugugaaaggaagcuccacugucacccuccaccucuucaccccccacucaccaguguccccuccacugucacauuguaacugaacuucaggauaauaaaguguuugccuccauggucuuugaauaaagccugaguaggaaggcggccgcucgagcaugcaucuaga

SEQ ID NO: 51 - RNA, 835 nt, Artificial Sequence
  Synthetic: 3UTR-007
acucaaucuaaauuaaaaaagaaagaaauuugaaaaaacuuucucuuugccauuucuucuucuucuuuuuuaacugaaagcugaauccuuccauuucuucugcacaucuacuugcuuaaauugugggcaaaagagaaaaagaaggauugaucagagcauugugcaauacaguuucauuaacuccuucccccgcucccccaaaaauuugaauuuuuuuuucaacacucuuacaccuguuauggaaaaugucaaccuuuguaagaaaaccaaaauaaaaauugaaaaauaaaaaccauaaacauuugcaccacuuguggcuuuugaauaucuuccacagagggaaguuuaaaacccaaacuuccaaagguuuaaacuaccucaaaacacuuucccaugagugugauccacauuguuaggugcugaccuagacagagaugaacugagguccuuguuuuguuuuguucauaauacaaaggugcuaauuaauaguauuucagauacuugaagaauguugauggugcuagaagaauuugagaagaaauacuccuguauugaguuguaucgugugguguauuuuuuaaaaaauuugauuuagcauucauauuuuccaucuuauucccaauuaaaaguaugcagauuauuugcccaaaucuucuucagauucagcauuuguucuuugccagucucauuuucaucuucuuccaugguuccacagaagcuuuguuucuugggcaagcagaaaaauuaaauuguaccuauuuuguauaugugagauguuuaaauaaauugugaaaaaaaugaaauaaagcauguuugguuuuccaaaagaacauau

SEQ ID NO: 52 - RNA, 297 nt, Artificial Sequence
  Synthetic: 3UTR-008
cgccgccgcccgggccccgcagucgagggucgugagcccaccccguccauggugcuaagcgggcccgggucccacacggccagcaccgcugcucacucggacgacgcccugggccugcaccucuccagcuccucccacgggguccccguagccccggcccccgcccagccccaggucuccccaggcccuccgcaggcugcccggccucccucccccugcagccaucccaaggcuccugaccuaccuggccccugagcucuggagcaagcccugacccaauaaaggcuuugaacccau

SEQ ID NO: 53 - RNA, 602 nt, Artificial Sequence
  Synthetic: 3UTR-009
ggggcuagagcccucuccgcacagcguggagacggggcaaggagggggguuauuaggauuggugguuuuguuuugcuuuguuuaaagccgugggaaaauggcacaacuuuaccucugugggagaugcaacacugagagccaaggggugggaguugggauaauuuuuauauaaaagaaguuuuuccacuuugaauugcuaaaaguggcauuuuuccuaugugcagucacuccucucauuucuaaaauagggacguggccaggcacgguggcucaugccuguaaucccagcacuuugggaggccgaggcaggcggcucacgaggucaggagaucgagacuauccuggcuaacacgguaaaacccugucucuacuaaaaguacaaaaaauuagcugggcgugguggugggcaccuguagucccagcuacucgggaggcugaggcaggagaaaggcaugaauccaagaggcagagcuugcagugagcugagaucacgccauugcacuccagccugggcaacaguguuaagacucugucucaaauauaaauaaauaaauaaauaaauaaauaaauaaauaaaaauaaagcgagauguugcccucaaa

SEQ ID NO: 54 - RNA, 785 nt, Artificial Sequence
  Synthetic: 3UTR-010
ggcccugccccgucggacugcccccagaaagccuccugcccccugccagugaaguccuucagugagccccuccccagccagcccuucccuggccccgccggauguauaaauguaaaaaugaaggaauuacauuuuauaugugagcgagcaagccggcaagcgagcacaguauuauuucuccauccccucccugccugcuccuuggcacccccaugcugccuucagggagacaggcagggagggcuuggggcugcaccuccuacccucccaccagaacgcaccccacugggagagcugguggugcagccuuccccucccuguauaagacacuuugccaaggcucuccccucucgccccaucccugcuugcccgcucccacagcuuccugagggcuaauucugggaagggagaguucuuugcugccccugucuggaagacguggcucugggugagguaggcgggaaaggauggaguguuuuaguucuugggggaggccaccccaaaccccagccccaacuccaggggcaccuaugagauggccaugcucaaccccccucccagacaggcccucccugucuccagggcccccaccgagguucccagggcuggagacuuccucugguaaacauuccuccagccuccccuccccuggggacgccaaggaggugggccacacccaggaagggaaagcgggcagccccguuuuggggacgugaacguuuuaauaauuuuugcugaauuccuuuacaacuaaauaacacagauauuguuauaaauaaaauugu

SEQ ID NO: 55 - RNA, 3001 nt, Artificial Sequence
  Synthetic: 3UTR-011
auauuaaggaucaagcuguuagcuaauaaugccaccucugcaguuuugggaacaggcaaauaaaguaucaguauacauggugauguacaucuguagcaaagcucuuggagaaaaugaagacugaagaaagcaaagcaaaaacuguauagagagauuuuucaaaagcaguaaucccucaauuuuaaaaaaggauugaaaauucuaaaugucuuucugugcauauuuuuuguguuaggaaucaaaaguauuuuauaaaaggagaaagaacagccucauuuuagauguaguccuguuggauuuuuuaugccuccucaguaaccagaaauguuuuaaaaaacuaaguguuuaggauuucaagacaacauuauacauggcucugaaauaucugacacaauguaaacauugcaggcaccugcauuuuauguuuuuuuuuucaacaaaugugacuaauuugaaacuuuuaugaacuucugagcuguccccuugcaauucaaccgcaguuugaauuaaucauaucaaaucaguuuuaauuuuuuaaauuguacuucagagucuauauuucaagggcacauuuucucacuacuauuuuaauacauuaaaggacuaaauaaucuuucagagaugcuggaaacaaaucauuugcuuuauauguuucauuagaauaccaaugaaacauacaacuugaaaauuaguaauaguauuuuugaagaucccauuucuaauuggagaucucuuuaauuucgaucaacuuauaauguguaguacuauauuaagugcacuugaguggaauucaacauuugacuaauaaaaugaguucaucauguuggcaagugauguggcaauuaucucuggugacaaaagaguaaaaucaaauauuucugccuguuacaaauaucaaggaagaccugcuacuaugaaauagaugacauuaaucugucuucacuguuuauaauacggauggauuuuuuuucaaaucaguguguguuuugaggucuuauguaauugaugacauuugagagaaaugguggcuuuuuuuagcuaccucuuuguucauuuaagcaccaguaaagaucaugucuuuuuauagaaguguagauuuucuuugugacuuugcuaucgugccuaaagcucuaaauauaggugaaugugugaugaauacucagauuauuugucucucuauauaauuaguuugguacuaaguuucucaaaaaauuauuaacacaugaaagacaaucucuaaaccagaaaaagaaguaguacaaauuuuguuacuguaaugcucgcguuuagugaguuuaaaacacacaguaucuuuugguuuuauaaucaguuucuauuuugcugugccugagauuaagaucuguguaugugugugugugugugugugcguuuguguguuaaagcagaaaagacuuuuuuaaaaguuuuaagugauaaaugcaauuuguuaauugaucuuagaucacuaguaaacucagggcugaauuauaccauguauauucuauuagaagaaaguaaacaccaucuuuauuccugcccuuuuucuucucucaaaguaguuguaguuauaucuagaaagaagcaauuuugauuucuugaaaagguaguuccugcacucaguuuaaacuaaaaauaaucauacuuggauuuuauuuauuuuugucauaguaaaaauuuuaauuuauauauauuuuuauuuaguauuaucuuauucuuugcuauuugccaauccuuugucaucaauuguguuaaaugaauugaaaauucaugcccuguucauuuuauuuuacuuuauugguuaggauauuuaaaggauuuuuguauauauaauuucuuaaauuaauauuccaaaagguuaguggacuuagauuauaaauuauggcaaaaaucuaaaaacaacaaaaaugauuuuuauacauucuauuucauuauuccucuuuuuccaauaagucauacaauugguagauaugacuuauuuuauuuuuguauuauucacuauaucuuuaugauauuuaaguauaaauaauuaaaaaaauuuauuguaccuuauagucugucaccaaaaaaaaaaaauuaucuguagguagugaaaugcuaauguugauuugucuuuaagggcuuguuaacuauccuuuauuuucucauuugucuuaaauuaggaguuuguguuuaaauuacucaucuaagcaaaaaauguauauaaaucccauuacuggguauauacccaaaggauuauaaaucaugcugcuauaaagacacaugcacacguauguuuauugcagcacuauucacaauagcaaagacuuggaaccaacccaaauguccaucaaugauagacuugauuaagaaaaugugcacauauacaccauggaauacuaugcagccauaaaaaaggaugaguucauguccuuuguagggacauggauaaagcuggaaaccaucauucugagcaaacuauugcaaggacagaaaaccaaacacugcauguucucacucauaggugggaauugaacaaugagaacacuuggacacaagguggggaacaccacacaccagggccugucaugggguggggggaguggggagggauagcauuaggagauauaccuaauguaaaugaugaguuaaugggugcagcacaccaacauggcacauguauacauauguagcaaaccugcacguugugcacauguacccuagaacuuaaaguauaauuaaaaaaaaaaagaaaacagaagcuauuuauaaagaaguuauuugcugaaauaaaugugaucuuucccauuaaaaaaauaaagaaauuuugggguaaaaaaacacaauauauuguauucuugaaaaauucuaagagaguggaugugaaguguucucaccacaaaagugauaacuaauugagguaaugcacauauuaauuagaaagauuuugucauuccacaauguauauauacuuaaaaauauguuauacacaauaaauacauacauuaaaaaauaaguaaaugua

SEQ ID NO: 56 - RNA, 1037 nt, Artificial Sequence
  Synthetic: 3UTR-012
cccacccugcacgccggcaccaaacccuguccucccaccccuccccacucaucacuaaacagaguaaaaugugaugcgaauuuucccgaccaaccugauucgcuagauuuuuuuuaaggaaaagcuuggaaagccaggacacaacgcugcugccugcuuugugcaggguccuccggggcucagcccugaguuggcaucaccugcgcagggcccucuggggcucagcccugagcuagugucaccugcacagggcccucugaggcucagcccugagcuggcgucaccugugcagggcccucuggggcucagcccugagcuggccucaccuggguuccccaccccgggcucuccugcccugcccuccugcccgcccucccuccugccugcgcagcuccuucccuaggcaccucugugcugcaucccaccagccugagcaagacgcccucucggggccugugccgcacuagccucccucuccucuguccccauagcugguuuuucccaccaauccucaccuaacaguuacuuuacaauuaaacucaaagcaagcucuucuccucagcuuggggcagccauuggccucugucucguuuugggaaaccaaggucaggaggccguugcagacauaaaucucggcgacucggccccgucuccugaggguccugcuggugaccggccuggaccuuggcccuacagcccuggaggccgcugcugaccagcacugaccccgaccucagagaguacucgcaggggcgcuggcugcacucaagacccucgagauuaacggugcuaaccccgucugcuccucccucccgcagagacuggggccuggacuggacaugagagccccuuggugccacagagggcugugucuuacuagaaacaacgcaaaccucuccuuccucagaauagugauguguucgacguuuuaucaaaggcccccuuucuauguucauguuaguuuugcuccuucuguguuuuuuucugaaccauauccauguugcugacuuuuccaaauaaagguuuucacuccucuc

SEQ ID NO: 57 - RNA, 577 nt, Artificial Sequence
  Synthetic: 3UTR-013
agaggccugccuccagggcuggacugaggccugagcgcuccugccgcagagcuggccgcgccaaauaaugucucugugagacucgagaacuuucauuuuuuuccaggcugguucggauuugggguggauuuugguuuuguuccccuccuccacucucccccacccccuccccgcccuuuuuuuuuuuuuuuuuuaaacugguauuuuaucuuugauucuccuucagcccucaccccugguucucaucuuucuugaucaacaucuuuucuugccucuguccccuucucucaucucuuagcuccccuccaaccuggggggcagugguguggagaagccacaggccugagauuucaucugcucuccuuccuggagcccagaggagggcagcagaaggggguggugucuccaaccccccagcacugaggaagaacggggcucuucucauuucaccccucccuuucuccccugcccccaggacugggccacuucuggguggggcagugggucccagauuggcucacacugagaauguaagaacuacaaacaaaauuucuauuaaauuaaauuuugugucucc

SEQ ID NO: 58 - RNA, 2212 nt, Artificial Sequence
  Synthetic: 3UTR-014
cucccuccaucccaaccuggcucccucccacccaaccaacuuuccccccaacccggaaacagacaagcaacccaaacugaacccccucaaaagccaaaaaaugggagacaauuucacauggacuuuggaaaauauuuuuuuccuuugcauucaucucucaaacuuaguuuuuaucuuugaccaaccgaacaugaccaaaaaccaaaagugcauucaaccuuaccaaaaaaaaaaaaaaaaaaagaauaaauaaauaacuuuuuaaaaaaggaagcuugguccacuugcuugaagacccaugcggggguaagucccuuucugcccguugggcuuaugaaaccccaaugcugcccuuucugcuccuuucuccacaccccccuuggggccuccccuccacuccuucccaaaucugucuccccagaagacacaggaaacaauguauugucugcccagcaaucaaaggcaaugcucaaacacccaaguggcccccacccucagcccgcuccugcccgcccagcacccccaggcccugggggaccugggguucucagacugccaaagaagccuugccaucuggcgcucccauggcucuugcaacaucuccccuucguuuuugagggggucaugccgggggagccaccagccccucacuggguucggaggagagucaggaagggccacgacaaagcagaaacaucggauuuggggaacgcgugucaaucccuugugccgcagggcugggcgggagagacuguucuguuccuuguguaacuguguugcugaaagacuaccucguucuugucuugaugugucaccggggcaacugccugggggcggggaugggggcaggguggaagcggcuccccauuuuauaccaaaggugcuacaucuaugugaugggugggguggggagggaaucacuggugcuauagaaauugagaugcccccccaggccagcaaauguuccuuuuuguucaaagucuauuuuuauuccuugauauuuuucuuuuuuuuuuuuuuuuuuuguggauggggacuugugaauuuuucuaaaggugcuauuuaacaugggaggagagcgugugcggcuccagcccagcccgcugcucacuuuccacccucucuccaccugccucuggcuucucaggccucugcucuccgaccucucuccucugaaacccuccuccacagcugcagcccauccucccggcucccuccuagucuguccugcguccucuguccccggguuucagagacaacuucccaaagcacaaagcaguuuuucccccuaggggugggaggaagcaaaagacucuguaccuauuuuguauguguauaauaauuugagauguuuuuaauuauuuugauugcuggaauaaagcauguggaaaugacccaaacauaauccgcaguggccuccuaauuuccuucuuuggaguugggggagggguagacauggggaaggggcuuuggggugaugggcuugccuuccauuccugcccuuucccuccccacuauucucuucuagaucccuccauaaccccacuccccuuucucucacccuucuuauaccgcaaaccuuucuacuuccucuuucauuuucuauucuugcaauuuccuugcaccuuuuccaaauccucuucuccccugcaauaccauacaggcaauccacgugcacaacacacacacacacucuucacaucugggguuguccaaaccucauacccacuccccuucaagcccauccacucuccacccccuggaugcccugcacuugguggcggugggaugcucauggauacugggagggugaggggaguggaacccgugaggaggaccugggggccucuccuugaacugacaugaagggucaucuggccucugcucccuucucacccacgcugaccuccugccgaaggagcaacgcaacaggagaggggucugcugagccuggcgagggucugggagggaccaggaggaaggcgugcucccugcucgcuguccuggcccugggggagugagggagacagacaccugggagagcuguggggaaggcacucgcaccgugcucuugggaaggaaggagaccuggcccugcucaccacggacugggugccucgaccuccugaauccccagaacacaaccccccugggcugggguggucuggggaaccaucgugcccccgccucccgccuacuccuuuuuaagcuu

SEQ ID NO: 59 - RNA, 729 nt, Artificial Sequence
  Synthetic: 3UTR-015
uuggccaggccugacccucuuggaccuuucuucuuugccgacaaccacugcccagcagccucugggaccucggggucccagggaacccaguccagccuccuggcuguugacuucccauugcucuuggagccaccaaucaaagagauucaaagagauuccugcaggccagaggcggaacacaccuuuauggcuggggcucuccgugguguucuggacccagccccuggagacaccauucacuuuuacugcuuuguagugacucgugcucuccaaccugucuuccugaaaaaccaaggcccccuucccccaccucuuccauggggugagacuugagcagaacaggggcuuccccaaguugcccagaaagacugucugggugagaagccauggccagagcuucucccaggcacagguguugcaccagggacuucugcuucaaguuuugggguaaagacaccuggaucagacuccaagggcugcccugagucugggacuucugccuccauggcuggucaugagagcaaaccguaguccccuggagacagcgacuccagagaaccucuugggagacagaagaggcaucugugcacagcucgaucuucuacuugccuguggggaggggagugacagguccacacaccacacugggucacccuguccuggaugccucugaagagagggacagaccgucagaaacuggagaguuucuauuaaaggucauuuaaacca

SEQ ID NO: 60 - RNA, 847 nt, Artificial Sequence
  Synthetic: 3UTR-016
uccuccgggaccccagcccucaggauuccugaugcuccaaggcgacugaugggcgcuggaugaaguggcacagucagcuucccugggggcuggugucauguugggcuccuggggcgggggcacggccuggcauuucacgcauugcugccaccccagguccaccugucuccacuuucacagccuccaagucuguggcucuucccuucuguccuccgaggggcuugccuucucucguguccagugaggugcucagugaucggcuuaacuuagagaagcccgcccccuccccuucuccgucugucccaagagggucugcucugagccugcguuccuagguggcucggccucagcugccuggguuguggccgcccuagcauccuguaugcccacagcuacuggaauccccgcugcugcuccgggccaagcuucugguugauuaaugagggcaugggguggucccucaagaccuuccccuaccuuuuguggaaccagugaugccucaaagacaguguccccuccacagcugggugccaggggcaggggauccucaguauagccggugaacccugauaccaggagccugggccucccugaaccccuggcuuccagccaucucaucgccagccuccuccuggaccucuuggcccccagccccuuccccacacagccccagaagggucccagagcugaccccacuccaggaccuaggcccagccccucagccucaucuggagccccugaagaccagucccacccaccuuucuggccucaucugacacugcuccgcauccugcuguguguccuguuccauguuccgguuccauccaaauacacuuucuggaacaaa

SEQ ID NO: 61 - RNA, 110 nt, Artificial Sequence
  Synthetic: 3UTR-017
gcuggagccucgguggccaugcuucuugccccuugggccuccccccagccccuccuccccuuccugcacccguacccccguggucuuugaauaaagucugagugggcggc

SEQ ID NO: 62 - RNA, 116 nt, Artificial Sequence
  Synthetic: 3UTR-018
uaauaggcuggagccucgguggccaugcuucuugccccuugggccuccccccagccccuccuccccuuccugcacccguacccccguggucuuugaauaaagucugagugggcggc

SEQ ID NO: 63 - RNA, 138 nt, Artificial Sequence
  Synthetic: 3UTR-018 + miR-122-5p binding site
uaauaggcuggagccucgguggccaugcuucuugccccuugggccuccccccagccccuccuccccuuccugcacccguaccccccaaacaccauugucacacuccaguggucuuugaauaaagucugagugggcggc

SEQ ID NO: 64 - RNA, 138 nt, Artificial Sequence
  Synthetic: 3UTR-018 + miR-122-3p binding site
uaauaggcuggagccucgguggccaugcuucuugccccuugggccuccccccagccccuccuccccuuccugcacccguacccccuauuuagugugauaauggcguuguggucuuugaauaaagucugagugggcggc

SEQ ID NO: 65 - protein, 198 aa, Mus musculus
  TNFSF4
MEGEGVQPLDENLENGSRPRFKWKKTLRLVVSGIKGAGMLLCFIYVCLQLSSSPAKDPPIQRLRGAVTRCEDGQLFISSYKNEYQTMEVQNNSVVIKCDGLYIIYLKGSFFQEVKIDLHFREDHNPISIPMLNDGRRIVFTVVASLAFKDKVYLTVNAPDTLCEHLQINDGELIVVQLTPGYCAPEGSYHSTVNQVPL

SEQ ID NO: 66 - RNA, 549 nt, Homo sapiens
  TNFSF4, ORF
auggaaaggguccaaccccuggaagagaaugugggaaaugcagccaggccaagauucgagaggaacaagcuauugcugguggccucuguaauucagggacuggggcugcuccugugcuucaccuacaucugccugcacuucucugcucuucagguaucacaucgguauccucgaauucaaaguaucaaaguacaauuuaccgaauauaagaaggagaaagguuucauccucacuucccaaaaggaggaugaaaucaugaaggugcagaacaacucagucaucaucaacugugauggguuuuaucucaucucccugaagggcuacuucucccaggaagucaacauuagccuucauuaccagaaggaugaggagccccucuuccaacugaagaaggucaggucugucaacuccuugaugguggccucucugacuuacaaagacaaagucuacuugaaugugaccacugacaauaccucccuggaugacuuccaugugaauggcggagaacugauucuuauccaucaaaauccuggugaauucuguguccuu

SEQ ID NO: 67 - RNA, 3484 nt, Homo sapiens
  TNFSF4, transcript variant 1, mRNA
ggcccugggaccuuugccuauuuucugauugauaggcuuuguuuugucuuuaccuccuucuuucuggggaaaacuucaguuuuaucgcacguuccccuuuuccauaucuucaucuucccucuacccagauugugaagauggaaaggguccaaccccuggaagagaaugugggaaaugcagccaggccaagauucgagaggaacaagcuauugcugguggccucuguaauucagggacuggggcugcuccugugcuucaccuacaucugccugcacuucucugcucuucagguaucacaucgguauccucgaauucaaaguaucaaaguacaauuuaccgaauauaagaaggagaaagguuucauccucacuucccaaaaggaggaugaaaucaugaaggugcagaacaacucagucaucaucaacugugauggguuuuaucucaucucccugaagggcuacuucucccaggaagucaacauuagccuucauuaccagaaggaugaggagccccucuuccaacugaagaaggucaggucugucaacuccuugaugguggccucucugacuuacaaagacaaagucuacuugaaugugaccacugacaauaccucccuggaugacuuccaugugaauggcggagaacugauucuuauccaucaaaauccuggugaauucuguguccuuugaggggcugauggcaauaucuaaaaccaggcaccagcaugaacaccaagcuggggguggacagggcauggauucuucauugcaagugaaggagccucccagcucagccacgugggaugugacaagaagcagauccuggcccucccgcccccaccccucagggauauuuaaaacuuauuuuauauaccaguuaaucuuauuuauccuuauauuuucuaaauugccuagccgucacaccccaagauugccuugagccuacuaggcaccuuugugagaaagaaaaaauagaugccucuucuucaagaugcauuguuucuauuggucaggcaauugucauaauaaacuuaugucauugaaaacgguaccugacuaccauuugcuggaaauuugacauguguguggcauuaucaaaaugaagaggagcaaggagugaaggagugggguuaugaaucugccaaaggugguaugaaccaaccccuggaagccaaagcggccucuccaagguuaaauugauugcaguuugcauauugccuaaauuuaaacuuucucauuugguggggguucaaaagaagaaucagcuugugaaaaaucaggacuugaagagagccgucuaagaaauaccacgugcuuuuuuucuuuaccauuuugcuuucccagccuccaaacauaguuaauagaaauuucccuucaaagaacugucuggggaugugaugcuuugaaaaaucuaaucagugacuuaagagagauuuucuuguauacagggagagugagauaacuuauugugaaggguuagcuuuacuguacaggauagcagggaacuggacaucucaggguaaaagucaguacggauuuuaauagccuggggaggaaaacacauucuuugccacagacaggcaaagcaacacaugcucauccuccugccuaugcugagauacgcacucagcuccaugucuuguacacacagaaacauugcugguuucaagaaaugaggugauccuauuaucaaauucaaucugaugucaaauagcacuaagaaguuauugugccuuaugaaaaauaaugaucucugucuagaaauaccauagaccauauauagucucacauugauaauugaaacuagaagggucuauaaucagccuaugccagggcuucaauggaauaguauccccuuauguuuaguugaaauguccccuuaacuugauauaauguguuaugcuuauggcgcuguggacaaucugauuuuucaugucaacuuuccagaugauuuguaacuucucugugccaaaccuuuuauaaacauaaauuuuugagauauguauuuuaaaauuguagcacauguuucccugacauuuucaauagaggauacaacaucacagaaucuuucuggaugauucuguguuaucaaggaauuguacugugcuacaauuaucucuagaaucuccagaaagguggagggcuguucgcccuuacacuaaauggucucaguuggauuuuuuuuuccuguuuucuauuuccucuuaaguacaccuucaacuauauucccaucccucuauuuuaaucuguuaugaaggaagguaaauaaaaaugcuaaauagaagaaauuguagguaagguaagaggaaucaaguucugaguggcugccaaggcacucacagaaucauaaucauggcuaaauauuuauggagggccuacuguggaccaggcacugggcuaaauacuuacauuuacaagaaucauucugagacagauauucaaugauaucuggcuucacuacucagaagauuguguguguguuuguguguguguguguguguguauuucacuuuuuguuauugaccauguucugcaaaauugcaguuacucagugagugauauccgaaaaaguaaacguuuaugacuauagguaauauuuaagaaaaugcaugguucauuuuuaaguuuggaauuuuuaucuauauuucucacagaugugcagugcacaugcaggccuaaguauauguuguguguguuguuugucuuugaugucaugguccccucucuuaggugcucacucgcuuugggugcaccuggccugcucuucccauguuggccucugcaaccacacagggauauuucugcuaugcaccagccucacuccaccuuccuuccaucaaaaauaugugugugugucucagucccuguaagucauguccuucacagggagaauuaacccuucgauauacauggcagaguuuugugggaaaagaauugaaugaaaagucaggagaucagaauuuuaaauuugacuuagccacuaacuagccauguaaccuugggaaagucauuucccauuucugggucuugcuuuucuuucuguuaaaugagaggaauguuaaauaucuaacaguuuagaaucuuaugcuuacaguguuaucugugaaugcacauauuaaaugucuauguucuuguugcuaugagucaaggaguguaaccuucuccuuuacuauguugaauguauuuuuuucuggacaagcuuacaucuuccucagccaucuuugugaguccuucaagagcaguuaucaauuguuaguuagauauuuucuauuuagagaaugcuuaagggauuccaaucccgauccaaaucauaauuuguucuuaaguauacugggcagguccccuauuuuaagucauaauuuuguauuuagugcuuuccuggcucucagagaguauuaauauugauauuaauaauauaguuaauaguaauauugcuauuuacauggaaacaaauaaaagaucucagaauucacuaaaaaaaaaaa

SEQ ID NO: 68 - RNA, 1609 nt, Mus musculus
  Mus musculus Tnfsf4, mRNA
auugcuuuuugucuccuguucugggaccuuuaucuucugacccgcaggcuugacuuugcccuuauuggcuccuuuguggugaagagcagucuucccccagguuccccgccacagcuguaucuccucugcaccccgacugcagagauggaaggggaagggguucaaccccuggaugagaaucuggaaaacggaucaaggccaagauucaaguggaagaagacgcuaaggcugguggucucugggaucaagggagcagggaugcuucugugcuucaucuaugucugccugcaacucucuuccucuccggcaaaggacccuccaauccaaagacucagaggagcaguuaccagaugugaggaugggcaacuauucaucagcucauacaagaaugaguaucaaacuauggaggugcagaacaauucgguugucaucaagugcgaugggcuuuauaucaucuaccugaagggcuccuuuuuccaggaggucaagauugaccuucauuuccgggaggaucauaaucccaucucuauuccaaugcugaacgauggucgaaggauugucuucacugugguggccucuuuggcuuucaaagauaaaguuuaccugacuguaaaugcuccugauacucucugcgaacaccuccagauaaaugauggggagcugauuguuguccagcuaacgccuggauacugugcuccugaaggaucuuaccacagcacugugaaccaaguaccacugugaauuccacucugaggguggacgggacacagguucuuucucgagagagaugagugcauccugcucaugagaugugacugaaugcagagccuacccuacuuccucacucagggauauuuaaaucaugucuuacauaacaguugaccucucauucccaggauugccuugagccugcuaagagcuguucugggaaugaaaaaaaaaauaaaugucucuucaagacacauugcuucugucggucagaagcucaucguaauaaacaucugccacugaaaauggcgcuugauugcuaucuucuagaauuuugauguugucaaaagaaagcaaaacauggaaagggugguguccaccggccaguaggagcuggagugcucucuucaagguuaaggugauagaaguuuacauguugccuaaaacugucucucaucucauggggggcuuggaaagaagauuaccccguggaaagcaggacuugaagaugacuguuuaagcaacaaggugcacucuuuuccuggccccugaauacacauaaaagacaacuuccuucaaagaacuaccuagggacuaugauacccaccaaagaaccacgucagcgaugcaaagaaaaccaggagagcuuuguuuauuuugcagaguauacgagagauuuuacccugagggcuauuuuuauuauacaggaugagagugaacuggaugucucaggauaaaggccaagaaggauuuuucacagucugagcaagacuguuuuuguagguucucucuccaaaacuuuuagguaaauuuuugauaauuuuaaaauuuuuaguuauauuuuuggaccauuuucaauagaagauugaaacauuuccagaugguuucauauccccacaag

SEQ ID NO: 69 - RNA, 737 nt, Homo sapiens
  mRNA sequence: Human OX40L with 5'-UTR, 3'-UTR, and miR-122 binding site
gggaaauaagagagaaaagaagaguaagaagaaauauaagagccaccauggaaaggguccaaccccuggaagagaaugugggaaaugcagccaggccaagauucgagaggaacaagcuauugcugguggccucuguaauucagggacuggggcugcuccugugcuucaccuacaucugccugcacuucucugcucuucagguaucacaucgguauccucgaauucaaaguaucaaaguacaauuuaccgaauauaagaaggagaaagguuucauccucacuucccaaaaggaggaugaaaucaugaaggugcagaacaacucagucaucaucaacugugauggguuuuaucucaucucccugaagggcuacuucucccaggaagucaacauuagccuucauuaccagaaggaugaggagccccucuuccaacugaagaaggucaggucugucaacuccuugaugguggccucucugacuuacaaagacaaagucuacuugaaugugaccacugacaauaccucccuggaugacuuccaugugaauggcggagaacugauucuuauccaucaaaauccuggugaauucuguguccuuugauaauaggcuggagccucgguggccaugcuucuugccccuugggccuccccccagccccuccuccccuuccugcacccguaccccccaaacaccauugucacacuccaguggucuuugaauaaagucugagugggcggc

SEQ ID NO: 70 - RNA, 782 nt, Artificial Sequence
  Synthetic: mRNA sequence: murine OX40L with 5'-UTR, 3'-UTR, and miR-122 binding site
gggaaauaagagagaaaagaagaguaagaagaaauauaagagccaccauggaaggggaagggguucaaccccuggaugagaaucuggaaaacggaucaaggccaagauucaaguggaagaagacgcuaaggcugguggucucugggaucaagggagcagggaugcuucugugcuucaucuaugucugccugcaacucucuuccucuccggcaaaggacccuccaauccaaagacucagaggagcaguuaccagaugugaggaugggcaacuauucaucagcucauacaagaaugaguaucaaacuauggaggugcagaacaauucgguugucaucaagugcgaugggcuuuauaucaucuaccugaagggcuccuuuuuccaggaggucaagauugaccuucauuuccgggaggaucauaaucccaucucuauuccaaugcugaacgauggucgaaggauugucuucacugugguggccucuuuggcuuucaaagauaaaguuuaccugacuguaaaugcuccugauacucucugcgaacaccuccagauaaaugauggggagcugauuguuguccagcuaacgccuggauacugugcuccugaaggaucuuaccacagcacugugaaccaaguaccacugugauaauaggcuggagccucgguggccaugcuucuugccccuugggccuccccccagccccuccuccccuuccugcacccguaccccccaaacaccauugucacacuccaguggucuuugaauaaagucugagugggcggc

SEQ ID NO: 71 - DNA, 1515 bp, Artificial Sequence; identical to SEQ ID NO: 19
  Synthetic: Codon optimized human IL-23 sequence

SEQ ID NO: 72 - DNA, 1515 bp, Artificial Sequence; identical to SEQ ID NO: 18
  Synthetic: Codon optimized human IL-23 sequence

SEQ ID NO: 73 - DNA, 1575 bp, Artificial Sequence
  Synthetic: Codon optimized murine IL-23 sequence
atgtgtcctcagaagctaaccatctcctggtttgccatcgttttgctggtgtctccactcatggccatgtgggagctggagaaagacgtttatgttgtagaggtggactggactcccgatgcccctggagaaacagtgaacctcacctgtgacacgcctgaagaagatgacatcacctggacctcagaccagagacatggagtcataggctctggaaagaccctgaccatcactgtcaaagagttcctagatgctggccagtacacctgccacaaaggaggcgagactctgagccactcacatctgctgctccacaagaaggaaaatggaatttggtccactgaaattttaaaaaatttcaaaaacaagactttcctgaagtgtgaagcaccaaattactccggacggttcacgtgctcatggctggtgcaaagaaacatggacttgaagttcaacatcaagagcagtagcagttcccctgactctcgggcagtgacatgtggaatggcgtctctgtctgcagagaaggtcacactggaccaaagggactatgagaagtattcagtgtcctgccaggaggatgtcacctgcccaactgccgaggagaccctgcccattgaactggcgttggaagcacggcagcagaataaatatgagaactacagcaccagcttcttcatcagggacatcatcaaaccagacccgcccaagaacttgcagatgaagcctttgaagaactcacaggtggaggtcagctgggagtaccctgactcctggagcactccccattcctacttctccctcaagttctttgttcgaatccagcgcaagaaagaaaagatgaaggagacagaggaggggtgtaaccagaaaggtgcgttcctcgtagagaagacatctaccgaagtccaatgcaaaggcgggaatgtctgcgtgcaagctcaggatcgctattacaattcctcatgcagcaagtgggcatgtgttccctgcagggtccgatccggaggcggagggagcggaggcggagggagcggaggcggagggagcgtgcctaggagtagcagtcctgactgggctcagtgccagcagctctctcggaatctctgcatgctagcctggaacgcacatgcaccagcgggacatatgaatctactaagagaagaagaggatgaagagactaaaaataatgtgccccgtatccagtgtgaagatggttgtgacccacaaggactcaaggacaacagccagttctgcttgcaaaggatccgccaaggtctggctttttataagcacctgcttgactctgacatcttcaaaggggagcctgctctactccctgatagccccatggagcaacttcacacctccctactaggactcagccaactcctccagccagaggatcacccccgggagacccaacagatgcccagcctgagttctagtcagcagtggcagcgcccccttctccgttccaagatccttcgaagcctccaggcctttttggccatagctgcccgggtctttgcccacggagcagcaactctgactgagcccttagtgccaacagct

SEQ ID NO: 74 - DNA, 1515 bp, Artificial Sequence
  Synthetic: Codon optimized human IL-23 sequence
atgtgccaccagcagctcgtgatcagctggttcagcctagtgttcctcgccagcccactcgtggccatctgggagctcaagaaggacgtctacgtagtagagctcgactggtacccggacgccccgggagagatggtcgtgctcacctgcgacaccccggaagaggacggcatcacctggaccctcgaccagagctccgaggtgctcggcagcggtaagaccctgaccatccaggtgaaggagttcggcgacgccggccaatacacctgccacaagggcggcgaggtgctgagccactccctgctgctcctgcataagaaggaggatggaatctggtccaccgacatcctcaaggaccagaaggagcctaagaacaagaccttcctccggtgcgaggccaagaactactcgggccgattcacctgttggtggctgactaccattagcaccgacctcaccttcagcgtcaagagcagcaggggcagcagcgaccctcagggcgtgacctgcggcgccgccaccctgagcgccgaaagggtgaggggcgacaacaaggagtacgaatatagcgtggagtgccaggaggacagcgcctgcccggccgccgaggagagcctgcctatcgaggtcatggtcgacgccgtgcacaagctgaagtacgagaactacaccagcagcttcttcatccgggacatcatcaagccggacccaccgaagaacctgcaactcaagccactgaagaacagccggcaggtggaggtgtcctgggagtaccctgacacctggagcacaccgcactcctatttctccctgaccttctgtgtgcaagtgcagggcaagagcaagagggagaagaaggaccgggtgttcaccgataagacctccgccaccgtgatctgcaggaagaacgcctccatcagcgtgagggcccaagacagatattacagcagctcatggtccgagtgggcctccgtcccatgctccggcggcggaggaggaggaagcagggccgtcccaggcggctctagccctgcctggacccaatgccagcagctgagccagaagctgtgcactctggcctggtccgcccacccgctggtgggccacatggatctgcgcgaggagggcgacgaggaaaccaccaacgacgtcccgcatatccagtgcggcgacggctgcgatccacagggcctgagggacaactcccagttctgcctgcagagaatccaccagggactgatcttctacgagaagctgctgggcagcgacatattcaccggcgaaccgagcctgctccctgacagcccggtgggccagctgcatgccagcctgctgggcctgtcacagctgctgcagccggagggccatcactgggagactcaacagatccctagcctcagccctagccagccgtggcagcggctgctgctcaggttcaagatcctgaggagcctgcaggccttcgtggcggtggccgcccgagtgttcgcccacggcgccgcgaccctgtccccg

SEQ ID NO: 75 - DNA, 1515 bp, Artificial Sequence
  Synthetic: Codon optimized human IL-23 sequence
atgtgccaccaacaactcgtgatctcctggttcagcctcgttttcctcgcaagcccactcgtggctatctgggaactcaagaaggacgtgtacgtggtggagctcgactggtacccggacgccccgggcgagatggtggtgctcacctgcgataccccggaggaggacggcatcacctggaccctcgaccagtccagcgaagtgctgggatccggcaagaccctgaccatccaggtgaaggagttcggcgatgccggccaatacacctgccacaagggcggcgaggtcctctcccacagcctgctgctgctccacaagaaggaggacggcatatggagcaccgacatcctgaaggaccagaaggaacctaagaacaagaccttcctgcgatgcgaggccaagaactacagcggcagattcacctgctggtggttaactaccataagcacagacctgaccttcagcgtaaagagcagcagaggcagcagcgacccgcagggcgtgacctgcggcgccgccaccctgtccgccgagcgggtgcggggcgacaacaaggagtatgagtactcagtggaatgccaggaggacagcgcctgcccggccgccgaggaaagcctgcctatcgaggtgatggtggacgccgtgcacaagctgaagtacgagaactacaccagcagcttcttcatcagggacatcatcaagccggacccgccgaagaacctgcaactgaagccgctgaagaacagccggcaagtggaggtgtcctgggagtacccggacacctggagcaccccgcatagctatttcagcctcaccttctgcgtgcaagtccagggcaagtccaagcgggagaagaaggacagggtgttcaccgacaagacttccgccactgtgatctgccgcaagaacgcgagcatctccgtgagggcgcaggataggtattatagcagcagctggtcggagtgggcctccgtgccttgctccggcggaggcggcggaggctcgagagccgtcccaggcggcagctccccagcctggacccagtgccagcagctgagccagaagctctgcaccctcgcctggagtgcccacccactggtgggccacatggacctccgcgaggaaggcgacgaggaaaccaccaatgacgtgccgcatatccagtgtggcgacggctgcgaccctcagggtctgagggataacagccagttctgcctccagcggatccatcagggcctgatcttctacgagaagctgctgggcagcgatatcttcaccggcgagccgtccctgctgccggacagcccggtgggccagctccacgccagcctgctgggcctcagccagctgctccagcctgaaggccaccattgggagactcagcagatcccgagcctgagcccgagccagccgtggcagagactgctgctccgtttcaagatcctcaggtcgctgcaggccttcgtggccgtggccgctagggtgttcgcccacggcgccgccaccctgtcccct

SEQ ID NO: 76 - DNA, 1515 bp, Artificial Sequence
  Synthetic: Codon optimized human IL-23 sequence
atgtgtcatcagcagctcgtgatcagctggttcagcctcgtgttcctcgcaagcccgctcgtcgccatctgggagctcaagaaggacgtgtacgttgtggagctcgactggtacccggacgccccgggcgagatggtggtgctcacctgcgacaccccggaggaggacggcatcacctggacgctggaccagagcagcgaggtgctgggcagcggcaagacgctgaccatccaggtgaaggaattcggcgatgccggccagtacacctgccacaagggcggcgaggttctgagccactcactgctgctcctccacaagaaggaggacggcatctggagcaccgacatcctgaaggaccagaaggagcctaagaacaagaccttcctgcggtgcgaggccaagaattacagcggacggttcacatgctggtggctgaccaccatcagcaccgacctgaccttcagcgtcaagtccagccggggctcaagcgacccgcagggcgtgacctgcggcgccgccaccctgagcgccgagagggtcagaggcgacaacaaggagtacgaatacagcgtggagtgtcaggaggactcggcctgcccggccgctgaggaatccctgccgatcgaagtaatggtggacgctgtgcacaagctgaagtacgagaactacaccagcagcttcttcatcagggacatcatcaagccagaccctcctaagaacctccagctgaagcctctgaagaacagccggcaggtggaggtgagctgggagtatccggacacctggtccaccccgcactcctacttcagccttacattctgcgtgcaggtgcagggcaagagcaagagggagaagaaggatagggtcttcaccgacaagaccagcgccaccgtcatctgcagaaagaacgcctctatctccgtcagggcccaggatcgctactacagcagcagctggagcgagtgggcttccgtcccttgctcaggtggcggtggcggcggcagcagggccgtcccgggtggcagctcgccggcctggacccagtgccagcaactctcgcagaagctgtgtaccctggcctggtcggcccatccgctggtgggccacatggacctgagggaggagggcgatgaggagacgaccaatgatgtgcctcacatccagtgtggcgacggctgcgaccctcaaggcctgagggacaatagccagttctgcctgcagaggatccatcagggcctgatcttctacgagaagctgctgggcagcgacattttcaccggcgagccgagcctcctgccggacagccctgtgggtcaactgcacgccagcctcctgggcctgtcccaactgctgcagccggagggccaccactgggaaacccagcagatcccaagcctgtccccgagccaaccgtggcagcgcctgctgctgcggttcaagatcctgagaagcctccaggctttcgtggcagtcgccgccagggtgttcgcccacggcgccgccaccctgtcccct

SEQ ID NO: 77 - DNA, 1515 bp, Artificial Sequence
  Synthetic: Codon optimized human IL-23 sequence
atgtgccaccagcagctcgtgattagctggttcagcctcgtgttcctcgccagcccgctcgtggccatctgggagcttaagaaggacgtgtacgtggtggagctcgactggtacccagacgcgccgggcgagatggtggtccttacctgcgacaccccggaagaggacggtattacctggaccctggatcagtctagcgaggtgctgggatcaggcaagaccctcaccatccaggtcaaggagttcggcgacgccggccagtatacgtgccacaagggaggcgaggtgctgagccattcgctgctgctcctgcacaagaaggaggatggcatctggagcaccgacattctcaaggaccagaaggagccgaagaacaagaccttcctcaggtgcgaagcaaagaattactccggacgcttcacctgctggtggctgacaaccatcagcaccgacctgacgttcagcgtcaagtccagcaggggcagcagcgacccgcagggcgtgacctgcggcgctgccaccctcagcgccgagcgagttaggggcgacaacaaggagtacgagtactccgtggagtgccaggaggactccgcttgcccggccgccgaggagtccctccctatcgaggtgatggtcgacgccgtgcacaagctgaagtatgagaactacaccagctcattcttcatcagagacatcatcaagccagacccgccgaagaacctccagctgaagcctctgaagaacagcaggcaggtggaggtgtcctgggagtacccggacacctggtccaccccgcactcctacttcagcctgaccttctgcgtgcaggtccaaggcaagagcaagcgggagaagaaggaccgcgtgttcaccgacaagacctccgccacggtcatatgcaggaagaacgccagcatcagcgtcagagcccaggatagatactactcgagctcctggtccgagtgggcgagcgtgccgtgcagcggcggaggcggtggcggctcccgagccgttccaggcggctctagcccggcatggacgcagtgccagcagctctcccagaagctgtgtaccctggcctggagcgcccacccactggtgggtcacatggacctgagggaggagggcgacgaggaaaccaccaatgatgtgccgcacatccagtgcggcgacggctgcgatcctcagggcctgcgggacaactcccagttctgcttacaaaggatccaccagggcctgatcttctacgagaagctcctgggctccgacatcttcaccggcgagccaagcctcctgccggacagtccggtgggccagctgcacgcctccctgctgggcctgagccaactgctgcagccggagggccaccactgggagacacagcagatacctagcctgtccccaagccagccttggcagcgcctgctgctgcgcttcaagatcctgagaagcttgcaggccttcgtggccgtggccgcccgggtgttcgcccacggcgccgcaaccctgagccca

SEQ ID NO: 78 - DNA, 1515 bp, Artificial Sequence
  Synthetic: Codon optimized human IL-23 sequence
atgtgtcaccagcagctcgtaatctcctggttcagcctcgtgttcctcgcctccccgctcgtggctatctgggagctcaagaaggacgtgtacgtggtcgagctcgactggtacccagacgcgccgggcgagatggtggtgctcacctgcgacacccctgaggaggacggcatcacctggaccttagaccagagctccgaggtgctcggcagcggcaagacactcactatccaagtgaaggagttcggcgatgccggccagtacacgtgccacaagggcggcgaggtgctgagccatagcctgctgctgctgcacaagaaggaagacggcatttggagcaccgacatcctgaaggaccagaaggagccgaagaacaagaccttcctgcgctgcgaggccaagaactactccggccgattcacctgttggtggctgacaaccatcagcactgacctgaccttctccgtcaagtcatcccgcggcagcagcgatccgcagggcgtcacctgcggagccgccaccctgtccgccgagagggtgcgcggcgacaacaaggagtacgagtactccgtggagtgccaggaggatagcgcctgcccagccgccgaggagtccctgccaatcgaggtgatggtggacgccgtgcataagctcaagtatgagaactacaccagcagcttcttcataagggacatcatcaagccggaccctccgaagaacctgcaactgaagccgctcaagaacagcaggcaagtggaggtgtcctgggaatacccggatacctggagcaccccgcactcctacttctccctgaccttctgcgttcaggtgcaaggaaagagcaagcgggagaagaaggaccgggtgttcaccgacaagaccagcgccaccgtgatctgccgcaagaatgccagcatcagcgtaagagcccaggacaggtactacagctcgtcctggtccgagtgggcctcggtgccgtgtagcggcggcggaggcggtggcagcagggccgtcccaggcggctcctcaccagcctggacacagtgccagcaactgagccagaagctgtgtaccctggcctggagcgcccacccgctggtgggccatatggacctgcgggaggagggcgacgaggagacgaccaacgatgtgccacacatccagtgcggtgatggatgcgatccacagggcctgagggacaacagccagttctgcctgcagagaatccaccagggcctgatcttctacgagaagctgctgggaagcgatattttcactggagaaccgagccttttgccggatagccctgtgggtcagctccacgccagcctgctgggtctgtcccagctgctccagccggagggccaccactgggaaacccagcagatcccgagcctgtccccaagccagccatggcaacggctgctgcttaggttcaagatcctgagaagcttacaggccttcgtggccgtggccgccagggtgttcgcccacggcgccgcgaccctgagcccg

SEQ ID NO: 79 - DNA, 1515 bp, Artificial Sequence
  Synthetic: Codon optimized human IL-23 sequence
atgtgccaccagcagttggtgatcagctggttcagcctcgtgttcctcgccagcccactcgtcgccatctgggagttgaagaaggacgtgtacgtggtggagctcgactggtacccggacgccccgggcgagatggtggtgctcacctgcgacaccccggaggaggacggcatcacgtggaccctggaccagagcagcgaggtcctgggcagcggcaagaccctcaccatccaggtgaaggagttcggcgacgccggccagtacacctgccacaagggcggagaagtgctgagccattccctgctgctgctgcataagaaggaggatggcatttggagcactgacatcctcaaggaccagaaggagccgaagaacaagacattcctgcgatgcgaggccaagaattacagcggtaggttcacctgctggtggcttacgaccatcagcacagacctgacgttctccgtgaagtccagcaggggcagcagcgatccgcagggcgtgacctgcggcgccgccaccctgagcgccgagcgggtgagaggagacaacaaggagtatgaatacagcgtggaatgtcaggaggactcggcctgcccggctgccgaggagagcctgccaatcgaggtgatggtggatgccgtgcacaagctgaagtacgagaactacaccagcagcttcttcatccgtgacatcatcaagccggacccgccgaagaacctgcagctgaagccgctcaagaactcccgacaggtggaagtgtcctgggagtatccagacacctggtcaaccccgcactcctacttctccctcacattctgcgtgcaggtgcagggcaagagcaagcgcgagaagaaggatagggtgttcaccgacaagacgagcgcgaccgtgatctgcaggaagaacgccagcatcagcgtgcgggcccaggacaggtactacagctcctcctggagcgaatgggcctccgtcccgtgctcaggcggtggcggcggcggctcgcgggccgtgccgggaggcagcagtcctgcatggacccagtgccaacagctgagccagaagctctgcacattggcctggagcgcccacccgctggtgggccacatggacctcagagaggagggcgacgaagaaaccaccaacgacgtgccgcacatccagtgcggcgacggctgcgaccctcagggtctgcgggacaatagccaattctgcctccagcgcatccatcagggcctgatcttctacgagaagcttctgggaagcgacatcttcaccggcgagccgagcctgctgccggacagcccggtgggccagctgcacgcctccctcctgggcctgagccagctgctgcaaccagagggccatcactgggaaacccagcagatccctagcctgagcccgagccagccgtggcagaggctgctcctgcggttcaagatcctcaggagcctgcaggccttcgtggccgtggcggcccgggtgttcgcccacggcgccgccaccctcagccca

SEQ ID NO: 80 - DNA, 1515 bp, Artificial Sequence
  Synthetic: Codon optimized human IL-23 sequence
atgtgccaccaacagctcgtgatcagctggttcagcctcgtgttcctcgccagcccgctcgtggccatctgggagctcaagaaggacgtgtacgtcgtcgaactcgactggtacccggacgcgccgggcgaaatggtggtgctaacctgcgacaccccggaagaggacggcatcacctggaccctggaccaatcaagcgaggtgctgggtagcggaaagaccctcaccatccaggtgaaggagttcggcgacgccggccaatacacgtgtcacaagggcggcgaggtgctgagccacagcctcctactgctgcacaagaaggaggacggtatctggagcaccgacatactgaaggaccagaaggagccgaagaacaagaccttcctgcgctgcgaggccaagaactactctggcaggttcacctgctggtggctcaccaccatcagcaccgacctgaccttcagcgtcaagagctcccggggcagtagcgatccgcagggcgtgacctgcggcgccgccaccctcagcgccgagcgcgtccgcggcgacaacaaggagtacgagtacagcgtggagtgccaggaggactccgcctgcccggccgccgaggagagcctcccgatcgaggtcatggtggacgccgtgcacaagctgaagtatgagaattacacctcctccttcttcatccgggatatcataaagccggacccgccgaagaacttacagctgaagcctctgaagaacagcaggcaggtggaggtgagctgggagtatccggacacctggagcaccccgcactcctatttcagcctgaccttctgcgtccaagtgcagggcaagagcaagagggagaagaaggacagggtgttcacggacaagaccagcgccaccgtaatctgtaggaagaacgccagcatcagcgtgcgagcccaggacaggtactactccagtagctggtccgagtgggcctccgtgccatgtagcggaggcggcggcggcggcagccgggccgtgccaggaggaagctctccggcctggacccagtgccaacagctgagccagaagctgtgcaccctggcctggagcgcccacccgctcgtgggccacatggatctgcgggaggagggcgacgaggaaactaccaacgacgtgccacacatccagtgcggcgacggctgcgacccacagggactgagggacaattcccagttctgcctccagcggatccaccagggcctgatcttctacgagaagctcctgggcagcgatatcttcaccggtgagccttccctgctgccggattcccctgtgggccagctccatgcctctctgctgggcctcagccagctgctgcaaccggagggacaccattgggagacgcagcaaatccctagcctgagcccgagccaaccatggcaaaggctcctgctgaggttcaagatcctgcgcagcctgcaggccttcgtggccgtcgccgcccgggtgttcgcccacggcgccgccacgctgagcccg

SEQ ID NO: 81 - DNA, 1515 bp, Artificial Sequence
  Synthetic: Codon optimized human IL-23 sequence
atgtgccaccagcagctcgtgataagctggttcagcctcgtcttcctcgcgagcccgctcgtcgccatctgggaactcaagaaggacgtgtacgtggtggagctcgattggtacccggacgccccgggtgagatggtggtcctcacctgcgacaccccggaggaggacggcatcacgtggactctggaccagagcagcgaagtgctcggctcgggtaagactctgaccatccaggtgaaggagttcggtgacgccggccagtacacctgccataagggcggagaggtgctctcccacagcctgctgctgctgcacaagaaggaagacggtatctggagcaccgatatcctgaaggaccagaaggagccgaagaacaagaccttcctgcggtgtgaggccaagaactacagcggcagattcacctgttggtggctgaccaccatctcgaccgacctgacattcagcgtgaagtcctccaggggtagcagcgacccgcagggcgtgacctgcggcgccgccaccctgtccgccgagcgggtgcgcggcgacaacaaggagtacgagtactccgtggagtgccaggaggacagcgcctgcccagcggcggaggagagcctccctatcgaagtgatggtggacgccgtacacaagctgaagtatgagaattacaccagcagcttcttcatccgggacataatcaagccggatccaccgaagaatctgcagctgaagccactgaagaacagccggcaggtggaggtgagctgggagtacccggacacctggtccacccctcacagctacttcagcctgaccttctgtgtgcaggtccagggcaagtccaagcgcgagaagaaggaccgagtgttcaccgacaagacctcggccaccgtgatctgccgtaagaacgcatctatcagcgtgcgggcccaggaccggtactacagctccagttggagcgaatgggccagcgtgccttgctccggcggcggcggcggcggaagcagggccgtgccgggcggcagctccccagcatggacccagtgccagcaactgagccagaagctgtgcaccctcgcctggtctgcccacccgctggtgggccacatggatctgcgggaggagggcgatgaggaaaccaccaacgacgtgccgcacatccagtgcggcgacggatgcgaccctcaaggcctgagagacaacagccagttctgcctgcagcgaatccaccagggcctgatcttctacgagaagctgctgggcagcgacatcttcaccggcgagccgagcctgctgccggacagcccggtgggccaactgcacgccagcctgctgggactgtcccaactgctgcagccggaaggccaccactgggagacacagcagatcccgagcctgagcccttcccagccgtggcagaggctgctgctgaggttcaagatcctccgttctctacaggccttcgtggccgtggcggccagagtgttcgcccacggcgccgctacgctctccccg

SEQ ID NO: 82 - DNA, 1515 bp, Artificial Sequence
  Synthetic: Codon optimized human IL-23 sequence
atgtgccaccagcagctcgtgatcagctggttctccttggtgttcctcgcatccccactcgtggccatctgggagctcaagaaggacgtgtacgtggtggagctcgactggtacccggacgccccaggcgagatggtggtgctcacctgtgacaccccggaggaggacggcatcacttggaccctggaccaaagctctgaggtcctgggctccggcaagacgctcaccatccaggtgaaggagttcggcgatgccggccagtacacctgccacaagggcggcgaggtgctgagccacagcctgctgctgctgcacaagaaggaggacggcatctggtccaccgatattcttaaggaccagaaggagccgaagaacaagacgttcctgcggtgcgaggccaagaactacagcggcagattcacctgctggtggctcactaccatcagcaccgacctgaccttcagcgtgaagtcctccaggggcagctccgacccgcagggagtcacctgcggcgccgccaccctgagtgcggaacgggtgagaggagacaacaaggagtacgagtactccgtggaatgtcaggaggacagcgcctgcccggccgccgaggagagcctgccgatcgaggtcatggtggacgccgtgcataagctgaagtacgagaactacaccagcagcttcttcatccgggacatcatcaagccggacccgccgaagaacctgcagctgaagccgctgaagaactcccgacaggtggaggttagctgggagtacccggacacctggagcaccccacacagctacttcagcctcaccttctgcgtgcaggtccagggcaagagcaagagggagaagaaggacagggtgttcaccgacaagaccagcgccacagtgatctgtagaaagaacgccagcatctccgtgcgcgcccaggaccgctactacagcagcagctggagcgagtgggctagcgtcccatgctccggtggcggtggcggcggcagcagagccgtgccgggcggcagcagcccagcctggacacagtgtcagcagctctcccagaagctgtgcaccctcgcctggagcgcccacccgctggtgggccacatggatctcagggaggagggcgacgaagaaaccaccaacgacgtgccgcacatccagtgtggcgatggatgcgacccgcagggcctgagggacaacagccagttctgcctgcagcggatccaccagggcctgatcttctatgagaagctgctgggctcagacattttcaccggcgaaccaagcctcctgccggacagcccggtgggacagctgcacgcctccctgctgggcctgagccagctgctccagccggagggccaccactgggaaacgcagcagatcccgagcctctccccaagccagccatggcagaggctcctgctccgcttcaagatcctgcggtccctgcaggccttcgtggccgtggccgcgagggtcttcgcccacggcgccgccaccctgagccct

SEQ ID NO: 83 - DNA, 1515 bp, Artificial Sequence
  Synthetic: Codon optimized human IL-23 sequence
atgtgccaccagcagctcgtgatcagctggttcagcctcgtgttccttgcctccccgctcgtggccatctgggagctcaagaaggacgtctacgtggtggagttggactggtatccagacgccccgggcgagatggtggtgcttacctgcgataccccagaggaggatggcattacctggaccctggaccagagcagcgaagtgctgggcagcggcaagaccctgaccatccaggtgaaggagttcggcgacgccggccaatacacctgccacaagggcggcgaggtgctgagccacagcctgctgcttctgcacaagaaggaggatggcatctggagcacagacatcctcaaggaccagaaggagccgaagaacaagaccttccttaggtgcgaggccaagaactactccggccggttcacctgctggtggctcaccaccatttccaccgacctgaccttcagcgtcaagagcagccggggatcctctgatccgcagggcgtgacctgcggcgccgccaccctgagcgccgaacgcgtgaggggcgacaacaaggagtacgagtattcagtcgagtgccaggaggacagcgcctgcccggccgccgaggagagcctgccgatcgaagtcatggtggacgccgtgcacaagctaaagtacgagaactacaccagctccttcttcatcagggacatcatcaagcctgacccgccaaagaacctgcagctgaagccgctgaagaactccaggcaggtggaggtcagctgggagtaccctgacacctggagcaccccgcactcctacttctcgctcaccttctgcgtgcaagtgcagggcaagtccaagagggagaagaaggaccgggtgttcaccgacaagaccagcgccaccgtgatatgcaggaagaacgccagcatctccgtccgggctcaggacaggtactacagctccagctggagcgaatgggcctccgtcccgtgcagcggcggcggtggcggcggtagccgtgccgtcccaggcggaagctcccctgcctggacacagtgtcagcagctgtcccagaagctgtgcaccctggcctggtccgcccatccgctcgtgggccatatggacctcagggaggagggcgacgaggaaacaaccaacgatgtgccgcatatccaatgcggcgacggctgcgatccgcagggcctgcgggataacagccaattctgcctgcagagaatccaccagggactgatcttctacgagaagctgctgggcagcgacatcttcacaggcgaacctagcctgctgccagactctcctgtgggtcagctgcacgccagcctgctgggcctctcccagctcctgcaaccggagggccaccactgggagacgcagcagatcccaagcctcagcccgtcccagccgtggcagaggctgctcctgcgcttcaagatcctgcgcagcctgcaggccttcgtcgcggtggcggcccgtgtgttcgcgcacggcgccgccaccctgtcccca

SEQ ID NO: 84 - DNA, 1515 bp, Artificial Sequence
  Synthetic: Codon optimized human IL-23 sequence
atgtgccaccagcagctcgtcatcagctggttcagcctcgtgttcctcgccagcccgctcgtggccatttgggagctcaagaaggacgtgtacgtggtcgagctcgattggtacccggacgccccaggagagatggtcgtcctcacctgcgacaccccggaggaggacggcatcacctggaccctcgaccaaagctccgaggtgctcggcagcggcaagaccctgacaatccaggtgaaggagttcggtgacgccggccagtacacctgccataagggcggcgaggtgctgagccacagcctgctgctgctgcacaagaaggaggacggcatctggtctaccgacatcctgaaggaccagaaggagccgaagaataagactttcctgaggtgcgaggccaagaactactccggccgcttcacctgttggtggctgaccactatctcgaccgacctgaccttcagcgtgaagtcctcgcggggctcctccgacccgcagggcgtgacctgcggcgccgccactctgtccgctgagagggtcaggggcgacaacaaggagtacgagtacagcgtcgagtgtcaggaggacagcgcctgcccggccgccgaggagtccctgccgattgaggtcatggtggacgcggtgcacaagctgaagtatgagaactataccagctccttcttcatccgggacattatcaagccggacccgccgaagaacctgcagctgaagccgctgaagaactcccgccaggtcgaggtgtcctgggagtatcctgacacctggtccaccccgcactcctacttcagcctgaccttctgcgtgcaggtgcaaggcaagagcaagcgagagaagaaggatagagtgttcaccgacaagaccagcgccaccgtgatttgcagaaagaacgccagcatctccgtgcgcgcccaggaccgctactacagcagcagctggtccgagtgggccagcgtgccatgcagcggcggaggcggaggcggtagccgcgccgtgccaggcggaagctccccggcgtggacccagtgccagcagctgagccagaagctctgcacactggcctggtccgcccatccactcgtgggccacatggacctccgggaggagggagacgaggaaacgacgaacgacgtgccgcacatccagtgcggcgacggctgcgacccgcagggactgcgggacaactcccagttctgcctgcagaggatccatcagggtctgatcttctacgagaagctgctgggcagcgacatcttcaccggcgaaccaagcctgctgcctgactcccctgtgggccagctgcacgcctccctgctgggcctgtcccagctgctccagccggagggccaccactgggaaacccaacaaatcccgagcctgagcccatcccagccgtggcagcgcctgctgctgaggttcaagatcctgcgctccctgcaggccttcgtcgccgtggccgccagagtattcgcccacggcgccgccaccctgagcccg

SEQ ID NO: 85 - DNA, 1515 bp, Artificial Sequence
  Synthetic: Codon optimized human IL-23 sequence
atgtgccaccagcagctcgtcatcagctggttctccctcgtgttcctcgcgagccctctcgtggccatctgggaactcaagaaggacgtgtacgtggtggagctcgactggtatccagacgccccgggcgaaatggtggtgctcacttgtgacaccccggaggaggacggtatcacctggaccctggaccagtccagcgaggtcctgggcagcggcaagacgctgaccatccaggtgaaggagttcggcgacgccggacagtacacctgccataagggcggagaggtgctcagccattccctgctcctgctgcacaagaaggaggacggcatatggagcacggacatactgaaggaccagaaggagcctaagaacaagaccttcctgagatgcgaggccaagaactactccggtcggttcacctgttggtggctcaccaccatctccaccgacctgaccttcagcgtgaagtcctccagaggctccagcgacccgcagggcgtcacctgcggcgccgccaccctgtccgccgagagggtgaggggcgacaataaggagtacgagtacagcgtggaatgtcaagaggatagcgcctgcccggccgccgaggaaagcctgccaatcgaggtgatggtggatgccgtgcacaagctgaagtatgagaactacaccagctccttcttcatcagggacatcatcaagccggacccgccgaagaacctgcagctcaagccactgaagaacagcagacaggtggaggtgtcctgggagtacccggacacatggagcaccccgcactcctacttctccctcaccttctgcgtccaggtgcagggcaagagcaagcgggagaagaaggacagggtgttcaccgataagacctccgccacagtgatctgccgcaagaacgcctccatcagcgtgagggcccaggacagatactacagctccagctggagcgagtgggccagcgtcccatgcagcggcggcggaggcggcggcagcagagccgtgccgggcggcagctccccagcatggacacagtgccagcagctgagccagaagctctgcaccctcgcctggtcggcccacccgctggtgggccacatggacctgcgcgaggaaggcgacgaggaaaccacgaacgacgtgccgcacatccagtgcggcgacggctgcgacccgcagggcctccgtgataacagccagttctgcctgcagaggatccaccagggcctgatcttctacgagaagctgctgggctccgacatcttcactggcgagccgagcctgctcccagatagcccagtgggacagctgcacgccagcctgctgggcctctcccagctgctccaaccggagggccatcactgggaaacccagcagatcccgagcctgtccccgagtcagccatggcagagactgctgctgaggttcaagatcctgcggtccctgcaggccttcgtggccgtggccgccagagtgttcgcccacggcgccgccaccctcagccca

SEQ ID NO: 86 - DNA, 1515 bp, Artificial Sequence
  Synthetic: Codon optimized human IL-23 sequence
atgtgccaccagcagctcgtgatcagctggttcagccttgtgttcttggccagcccccttgtggccatctgggagttaaagaaggacgtgtacgtggtggagttagactggtaccccgacgcccccggcgagatggtggtgctcacctgcgacacccccgaggaggacggcatcacctggaccctggaccagagcagcgaggtgctgggcagcggcaagaccctgaccatccaggtgaaggagttcggcgacgccggccagtacacctgccacaagggcggcgaagtgctgagccacagcctgctgctcctgcacaagaaggaagatggcatctggagcaccgacatcctgaaggaccagaaggagcccaagaacaagaccttcctgcggtgcgaggccaagaactacagcggccggttcacctgctggtggctgaccaccatcagcaccgatctgaccttcagcgtcaagtccagccggggcagcagcgacccccagggcgtgacctgtggcgccgccaccctgagcgccgagcgggtgcggggcgacaacaaggagtacgagtacagcgtggagtgccaggaggacagcgcctgccccgccgccgaggagagcctgcccatcgaggtgatggtggacgccgtgcacaagctgaagtacgagaactacacctccagcttcttcatccgggacatcatcaagcccgacccccctaagaacctgcagctgaagcccctgaagaacagccggcaggtggaggtgagctgggagtacccagacacatggagcacaccccacagctacttctccttgaccttctgcgtgcaggtgcagggcaagagcaagcgggagaagaaggatcgggtgttcaccgacaagaccagcgccaccgtgatctgccggaagaacgccagcatcagcgtgcgggcccaggaccggtactactcttcttcgtggagcgagtgggccagcgtgccctgcagcggcggcggaggaggcggcagcagagccgtgccgggcggcagttcccccgcctggactcagtgccagcaactgagccagaagctgtgcaccctggcctggagcgcccacccactggtgggccacatggacctgagagaggagggcgacgaggagacgaccaacgacgtgccccacatccagtgcggcgacggctgcgacccacagggtctgcgagacaacagccagttctgcctgcagaggatccaccagggcttgatcttctacgagaagctgctgggaagcgacatcttcaccggcgagccttccctgctgcccgacagccccgtcggccagctgcacgccagcctcctgggcctgtcccagctgctccagcccgagggccaccactgggaaacccagcagatcccaagcctgagccccagccagccctggcagagactgctgctgcggttcaagatcctgcggagcctgcaggccttcgtggccgtggccgccagagtcttcgcccacggagccgccacactaagcccc

SEQ ID NO: 87 - DNA, 1515 bp, Artificial Sequence
  Synthetic: Codon optimized human IL-23 sequence
atgtgccaccagcagcttgtgatcagctggttcagccttgtgttcctcgccagccccttagtggccatctgggagctcaagaaggacgtgtacgtggtggagctcgactggtaccccgacgcccccggcgagatggtggtgctaacctgcgacacccccgaggaggacggcatcacctggaccctggaccagagcagcgaggtgctgggcagcggcaagaccctgaccatccaggtgaaggagttcggcgacgccggccagtacacctgccacaagggcggcgaggtcctgagccacagcctgttgctcctgcacaagaaggaagacggtatctggagcaccgacatcctgaaggaccagaaggagcccaagaacaagaccttcctgcggtgcgaggccaagaactacagcggccggttcacctgctggtggctgaccaccatctccaccgacctgaccttcagcgtgaagtccagccggggcagcagcgacccccagggcgtgacatgcggcgccgccaccctgagcgccgagcgggtgcggggcgacaacaaggagtacgagtacagcgtggagtgccaggaggacagcgcctgccccgccgccgaggagagcctgcccatcgaggtgatggtggacgccgtgcacaagctgaagtacgagaactacacaagcagcttcttcatccgggacatcatcaagcccgacccccctaagaacctgcagctgaagcccctgaagaacagccggcaggtggaggtgagctgggagtaccctgacacctggtctaccccccacagctacttcagcctcaccttctgcgtgcaggtgcagggcaagagcaagcgggagaagaaggatcgggtgttcaccgacaagaccagcgccaccgtgatctgccggaagaacgccagcatcagcgtgcgggcccaggaccggtactacagcagctcttggagcgagtgggccagcgtgccctgcagcggcggtggcggcggcggaagcagagccgtgccaggcggctctagccccgcatggacccagtgtcaacagctgagccagaagctgtgcaccctggcctggagcgcccaccctttggtgggccacatggacctgagagaggagggcgacgaggaaacgaccaacgacgtgccccacatccagtgcggcgacggctgtgaccctcagggcctgcgggacaacagccagttctgcctgcagaggatccaccagggattgatcttctacgagaagctcctgggctctgacatcttcaccggcgagccaagcctgctccccgacagccccgtgggacagctgcacgcctccctgctgggcctgtcacagctccttcagcccgagggccaccactgggagacacagcagatcccatctctgagccccagccagccctggcagagactgttgctgcggttcaagatcctgcggagcctgcaggccttcgtggccgtggccgccagggtgttcgcccacggagcagccacactgtccccc

SEQ ID NO: 88 - DNA, 1515 bp, Artificial Sequence
  Synthetic: Codon optimized human IL-23 sequence
atgtgccaccagcagcttgtgatcagctggttcagcttagtgttcctcgccagccccttagtggccatctgggagctcaagaaggacgtgtacgtggtggagcttgactggtaccccgacgcccccggcgagatggtggtgctcacctgcgacacccccgaggaggacggcatcacctggaccctggaccagagcagcgaggtgctgggcagcggcaagaccctgaccatccaggtgaaggagttcggcgacgccggccagtacacctgccacaagggcggcgaggttcttagccacagcctgctgcttctgcacaagaaggaggatggcatctggagcaccgacatcctgaaggaccagaaggagcccaagaacaagaccttcctgcggtgcgaggccaagaactacagcggccggttcacctgctggtggctgaccaccatctctaccgacctgaccttcagcgttaagagcagccggggcagcagcgacccccagggcgtaacctgcggcgccgccaccctgagcgccgagcgggtgcggggcgacaacaaggagtacgagtacagcgtggagtgccaggaggacagcgcctgccccgccgccgaggagagcctgcccatcgaggtgatggtggacgccgtgcacaagctgaagtacgagaactatacctctagcttcttcatccgggacatcatcaagcccgaccccccaaagaacctgcagctgaagcccctgaagaacagccggcaggtggaggtgagctgggagtaccctgacacatggagcacaccccacagctacttcagtctgacattctgcgtgcaggtgcagggcaagagcaagcgggagaagaaggatcgggtgttcaccgacaagaccagcgccaccgtgatctgccggaagaacgccagcatcagcgtgcgggcccaggaccggtactacagcagctcctggagcgagtgggccagcgtgccctgcagcggcggcggaggaggcggcagcagagccgtgccaggcggctcctctcccgcgtggacccagtgccagcagttgagccagaagctgtgcaccctggcatggtccgcccacccactggtgggccacatggacctcagggaggagggcgacgaggagacaaccaacgacgtgccccacatccagtgcggcgacggctgcgacccacagggcctgagagacaacagccagttctgtctgcagagaatccaccagggactgatcttctacgagaagctgctcggctccgacatcttcaccggcgagcctagcctcctgcccgacagccccgtgggacagctgcacgccagtttgttgggcctgtcacaactgctgcagcccgagggccaccactgggagacgcagcagatccctagcctgagccccagccagccctggcagcggttactgctgcggttcaagatcctgcggagcctgcaggccttcgtggccgtggccgcccgcgtgttcgcccacggagcggccacactgagcccc

SEQ ID NO: 89 - DNA, 1515 bp, Artificial Sequence
  Synthetic: Codon optimized human IL-23 sequence
atgtgccaccagcagctcgtgatcagctggttcagccttgtgttcctcgccagccccctcgtggccatctgggagctcaagaaggacgtgtacgtcgtcgagctcgactggtaccccgacgcccccggcgagatggtcgtcctcacctgcgacacccccgaggaggacggcatcacctggaccctcgaccagtcctccgaggtcctcggctccggcaagaccctcaccatccaggtcaaggagttcggcgacgccggccagtacacctgccacaagggcggagaggttctgtcccactccctgctgctactccacaagaaggaggatggcatctggtccaccgacatcctcaaggaccagaaggagcccaagaacaagaccttcctccgctgcgaggccaagaactactccggccgcttcacctgctggtggctcaccaccatctccacagacctcaccttctccgtcaagtcctcccgcggctcctccgacccccagggcgttacctgcggcgccgccaccctctccgccgagcgcgtccgcggcgacaacaaggagtacgagtactccgtcgagtgccaggaggactccgcctgccccgccgccgaggagtccctccccatcgaggtcatggtcgacgccgtccacaagctcaagtacgagaactacaccagctccttcttcatccgcgacatcatcaagcctgaccctcctaagaatctccagctcaagcccctcaagaactcccgccaggtcgaggtgtcctgggaatatccagacacctggagcaccccccactcctacttctccctgaccttctgcgtccaggtccagggcaagtccaagcgcgagaagaaggatcgcgtcttcaccgacaagacatccgccaccgtcatctgccgcaagaacgcctccatctccgtccgcgcccaggaccgctactactcctcctcttggtccgagtgggcctccgtcccctgctccggcggaggcggcggtggatcccgcgccgtccctggcggcagctccccagcttggacccagtgtcagcagctctcccagaagctctgcaccctcgcctggagcgcccaccccctcgtcggccacatggacctcagggaggagggcgacgaggagacaaccaacgacgtcccccacatccagtgcggcgacggctgcgacccacagggacttagagacaactcccagttctgcctccagcgcatccaccagggcctcatcttctacgagaagcttttgggatccgacatcttcactggcgagcctagcctgctgccggactcccctgtgggccagctccacgcgtctctgctgggcctgagtcagctcctccagcccgagggccaccactgggaaacccagcagatcccttccttgtccccctcccagccctggcagcgcctcctgctgcggttcaagatcctgagatccctccaggccttcgtcgccgtcgccgcccgggtcttcgcccatggcgctgctacactgagcccc

SEQ ID NO: 90 - DNA, 1515 bp, Artificial Sequence
  Synthetic: Codon optimized human IL-23 sequence
atgtgccaccagcagctcgtgatcagctggttcagcctcgtgttcctagccagcccccttgtggccatctgggagctcaagaaggacgtgtacgtcgtcgagctcgactggtaccccgacgcccccggcgagatggtcgtcctcacctgcgacacccccgaggaggacggcatcacctggaccctcgaccagtcctccgaggtcctcggctccggcaagaccctcaccatccaggtcaaggagttcggcgacgccggccagtacacctgccacaagggcggcgaggtgctgtcccactccctgctgctgctccacaagaaggaggatggcatctggtccaccgacatcctcaaggaccagaaggagcccaagaacaagaccttcctccgctgcgaggccaagaactactccggccgcttcacctgctggtggctcaccaccatcagcaccgacctcaccttctccgtcaagtcctcccgcggctcctccgacccccagggcgtgacatgcggcgccgccaccctctccgccgagcgcgtccgcggcgacaacaaggagtacgagtactccgtcgagtgccaggaggactccgcctgccccgccgccgaggagtccctccccatcgaggtcatggtcgacgccgtccacaagctcaagtacgagaactacaccagtagcttcttcatccgcgacatcatcaagcctgaccctccaaagaacctccagctcaagcccctcaagaactcccgccaggtcgaagtgtcctgggagtacccagacacctggtcaactccccactcctacttcagccttacgttctgcgtccaggtccagggcaagtccaagcgcgagaagaaggatcgcgtcttcaccgacaagacttccgccaccgtcatctgccgcaagaacgcctccatctccgtccgcgcccaggaccgctactacagctcctcttggtccgagtgggcctccgtcccctgctccggaggcggtggcggcggatcccgcgccgtcccaggcggaagctcccccgcatggacccagtgtcagcagctctcccagaagctctgcaccctcgcctggtccgcccaccccctcgtcggccacatggacctgcgcgaggagggcgacgaggagacaaccaacgacgtcccccacatccagtgcggcgacggctgcgatccacagggcctgagggacaactcccagttctgcctccagcgcatccaccagggactcatcttctacgagaagctgctgggaagcgacatattcaccggcgagccttccttgctgccagactcccctgtgggccagctccacgcctccctcctgggcctctcccaactgctccagcccgagggccaccactgggagacacagcagatcccatccctgtccccctcccagccctggcagcgcctgctactgcgcttcaagatcctgagatccctccaggccttcgtcgccgtcgccgccagagtgttcgcccatggagccgccacactgagcccc

SEQ ID NO: 91 - DNA, 1515 bp, Artificial Sequence
  Synthetic: Codon optimized human IL-23 sequence
atgtgccaccagcagctggtgatcagctggttcagcctggtgttcctggccagccccctggtggccatctgggagctgaagaaggacgtgtacgtggtggagctggactggtaccccgacgcccccggcgagatggtggtgctgacctgcgacacccccgaggaggacggcatcacctggaccctggaccagagcagcgaggtgctgggcagcggcaagaccctgaccatccaggtgaaggagttcggcgacgccggccagtacacctgccacaagggcggcgaggtgctgagccacagcctgctgctgctgcacaagaaggaggacggcatctggagcaccgacatcctgaaggaccagaaggagcccaagaacaagaccttcctgcggtgcgaggccaagaactacagcggccggttcacctgctggtggctgaccaccatcagcaccgacctgaccttcagcgtgaagagcagccggggcagcagcgacccccagggcgtgacctgcggcgccgccaccctgagcgccgagcgggtgcggggcgacaacaaggagtacgagtacagcgtggagtgccaggaggacagcgcctgccccgccgccgaggagagcctgcccatcgaggtgatggtggacgccgtgcacaagctgaagtacgagaactacaccagcagcttcttcatccgggacatcatcaagcccgacccccccaagaacctgcagctgaagcccctgaagaacagccggcaggtggaggtgagctgggagtaccccgacacctggagcaccccccacagctacttcagcctgaccttctgcgtgcaggtgcagggcaagagcaagcgggagaagaaggaccgggtgttcaccgacaagaccagcgccaccgtgatctgccggaagaacgccagcatcagcgtgcgggcccaggaccggtactacagcagcagctggagcgagtgggccagcgtgccctgcagcggcggcggcggcggcggcagccgggccgtgcccggcggcagcagccccgcctggacccagtgccagcagctgagccagaagctgtgcaccctggcctggagcgcccaccccctggtgggccacatggacctgcgggaggagggcgacgaggagaccaccaacgacgtgccccacatccagtgcggcgacggctgcgacccccagggcctgcgggacaacagccagttctgcctgcagcggatccaccagggcctgatcttctacgagaagctgctgggcagcgacatcttcaccggcgagcccagcctgctgcccgacagccccgtgggccagctgcacgccagcctgctgggcctgagccagctgctgcagcccgagggccaccactgggagacccagcagatccccagcctgagccccagccagccctggcagcggctgctgctgcggttcaagatcctgcggagcctgcaggccttcgtggccgtggccgcccgggtgttcgcccacggcgccgccaccctgagcccc

SEQ ID NO: 92 - DNA, 1515 bp, Artificial Sequence
  Synthetic: Codon optimized human IL-23 sequence
atgtgccaccagcagctggtgatcagctggttcagcctggtgttcctggccagccccctggtggccatctgggagctgaagaaggacgtgtacgtggtggagctggactggtacccggacgcgccgggggagatggtggtgctgacgtgcgacacgccggaggaggacgggatcacgtggacgctggaccagagcagcgaggtgctggggagcgggaagacgctgacgatccaggtgaaggagttcggggacgcggggcagtacacgtgccacaaggggggggaggtgctgagccacagcctgctgctgctgcacaagaaggaggacgggatctggagcacggacatcctgaaggaccagaaggagccgaagaacaagacgttcctgaggtgcgaggcgaagaactacagcgggaggttcacgtgctggtggctgacgacgatcagcacggacctgacgttcagcgtgaagagcagcagggggagcagcgacccgcagggggtgacgtgcggggcggcgacgctgagcgcggagagggtgaggggggacaacaaggagtacgagtacagcgtggagtgccaggaggacagcgcgtgcccggcggcggaggagagcctgccgatcgaggtgatggtggacgcggtgcacaagctgaagtacgagaactacacgagcagcttcttcatcagggacatcatcaagccggacccgccgaagaacctgcagctgaagccgctgaagaacagcaggcaggtggaggtgagctgggagtacccggacacgtggagcacgccgcacagctacttcagcctgacgttctgcgtgcaggtgcaggggaagagcaagagggagaagaaggacagggtgttcacggacaagacgagcgcgacggtgatctgcaggaagaacgcgagcatcagcgtgagggcgcaggacaggtactacagcagcagctggagcgagtgggcgagcgtgccgtgcagcggggggggggggggggggagcagggcggtgccgggggggagcagcccggcgtggacgcagtgccagcagctgagccagaagctgtgcacgctggcgtggagcgcgcacccgctggtggggcacatggacctgagggaggagggggacgaggagacgacgaacgacgtgccgcacatccagtgcggggacgggtgcgacccgcaggggctgagggacaacagccagttctgcctgcagaggatccaccaggggctgatcttctacgagaagctgctggggagcgacatcttcacgggggagccgagcctgctgccggacagcccggtggggcagctgcacgcgagcctgctggggctgagccagctgctgcagccggaggggcaccactgggagacgcagcagatcccgagcctgagcccgagccagccgtggcagaggctgctgctgaggttcaagatcctgaggagcctgcaggcgttcgtggcggtggcggcgagggtgttcgcgcacggggcggcgacgctgagcccg

SEQ ID NO: 93 - DNA, 1515 bp, Artificial Sequence
  Synthetic: Codon optimized human IL-23 sequence
atgtgccaccagcagctggtgatcagctggttcagcctggtgttcctggccagccccctggtggccatctgggagctgaagaaggacgtgtacgtcgtcgagctcgactggtaccccgacgcccccggcgagatggtcgtcctcacctgcgacacccccgaggaggacggcatcacctggaccctcgaccagtcctccgaggtcctcggctccggcaagaccctcaccatccaggtcaaggagttcggcgacgccggccagtacacctgccacaagggcggcgaggtcctctcccactccctcctcctcctccacaagaaggaggacggcatctggtccaccgacatcctcaaggaccagaaggagcccaagaacaagaccttcctccgctgcgaggccaagaactactccggccgcttcacctgctggtggctcaccaccatctccaccgacctcaccttctccgtcaagtcctcccgcggctcctccgacccccagggcgtcacctgcggcgccgccaccctctccgccgagcgcgtccgcggcgacaacaaggagtacgagtactccgtcgagtgccaggaggactccgcctgccccgccgccgaggagtccctccccatcgaggtcatggtcgacgccgtccacaagctcaagtacgagaactacacctcctccttcttcatccgcgacatcatcaagcccgacccccccaagaacctccagctcaagcccctcaagaactcccgccaggtcgaggtctcctgggagtaccccgacacctggtccaccccccactcctacttctccctcaccttctgcgtccaggtccagggcaagtccaagcgcgagaagaaggaccgcgtcttcaccgacaagacctccgccaccgtcatctgccgcaagaacgcctccatctccgtccgcgcccaggaccgctactactcctcctcctggtccgagtgggcctccgtcccctgctccggcggcggcggcggcggctcccgcgccgtccccggcggctcctcccccgcctggacccagtgccagcagctctcccagaagctctgcaccctcgcctggtccgcccaccccctcgtcggccacatggacctccgcgaggagggcgacgaggagaccaccaacgacgtcccccacatccagtgcggcgacggctgcgacccccagggcctccgcgacaactcccagttctgcctccagcgcatccaccagggcctcatcttctacgagaagctcctcggctccgacatcttcaccggcgagccctccctcctccccgactcccccgtcggccagctccacgcctccctcctcggcctctcccagctcctccagcccgagggccaccactgggagacccagcagatcccctccctctccccctcccagccctggcagcgcctcctcctccgcttcaagatcctccgctccctccaggccttcgtcgccgtcgccgcccgcgtcttcgcccacggcgccgccaccctctccccc

SEQ ID NO: 94 - DNA, 516 bp, Artificial Sequence; identical to SEQ ID NO: 17
  Synthetic: Codon optimized hIGKV4-hIL-36g

SEQ ID NO: 95 - DNA, 516 bp, Artificial Sequence
  Synthetic: Codon optimized hIGKV4-hIL-36g
atggtgctccagacccaggtgttcatctccttgctcttgtggatcagtggcgcttacggatcaatgtgcaagcctattaccggcaccatcaacgacttaaaccagcaggtttggaccctccagggccagaacctcgttgccgtgcctcgcagcgacagcgtgacccctgtcaccgtggccgtgatcacgtgtaagtaccctgaagcactggagcagggcagaggcgacccaatttatctcggaatccagaacccggagatgtgcctgtactgcgagaaggtgggcgaacagcctaccctgcagctgaaggagcagaagatcatggatctgtatggacagcctgagccggtgaagccgttcctgttctacagagcgaagactggaaggacaagcaccctagagagcgtcgccttcccggactggttcatcgccagctcaaagagggatcagcctatcattctgacgtcagagcttggcaagagctacaacaccgccttcgagcttaatatcaacgac

SEQ ID NO: 96 - DNA, 516 bp, Artificial Sequence
  Synthetic: Codon optimized hIGKV4-hIL-36g
atggtgcttcagacccaggtgttcatcagcctactcctctggatcagcggcgcctacggcagcatgtgcaagcccatcaccggcaccatcaacgacttaaaccagcaggtgtggaccctccagggccagaaccttgtggccgtgccccggagcgacagcgtgaccccggtgaccgttgctgtgatcacctgcaagtaccccgaggccctggagcagggccggggcgaccccatctacctgggcatccagaaccccgagatgtgcctgtactgcgagaaggtgggcgagcagcccactttgcagctgaaggagcagaagatcatggacctgtacggccagcccgagcccgtgaagcccttcctgttctaccgggccaagaccggccggaccagcaccctggagagcgtggccttccccgactggttcatcgccagcagcaagcgggaccagccgatcatcctgaccagcgagctgggcaagagctacaacaccgccttcgagctgaatatcaatgac

SEQ ID NO: 97 - DNA, 516 bp, Artificial Sequence
  Synthetic: Codon optimized hIGKV4-hIL-36g
atggtgctccagacgcaggtgttcatcagcttgcttctttggatcagcggagcctacggctccatgtgcaagcctatcacaggcaccatcaacgacttaaaccagcaggtgtggaccctccagggtcagaacttagtggccgtgcctcggagcgacagcgtcacgcctgtgaccgtggccgtaataacctgtaagtatcctgaggccctggaacagggcaggggagatccaatatacctgggcatccagaaccctgagatgtgtctctactgcgagaaggtgggcgaacagcctaccttgcagctgaaggagcagaagataatggacctgtacggacagccagaaccagtcaagccgttcctgttctatagagccaagaccggtagaacctccacgctcgagtccgtggcattccctgactggttcatcgcctccagcaagcgcgaccagccgatcatactgacctctgagttgggcaagagctataacaccgccttcgagctgaatatcaatgac

SEQ ID NO: 98 - DNA, 516 bp, Artificial Sequence
  Synthetic: Codon optimized: hIGKV4-hIL-36g
atggtgcttcagacccaggtgttcatcagcttgctcctctggatcagcggcgcctacggcagcatgtgcaagcccatcaccggcaccatcaacgacctcaaccagcaggtctggaccctccagggccagaacctcgtcgccgtgcctcgctccgactccgtcacccctgtcacggtggccgtgatcacctgcaagtaccccgaggccctcgagcagggccgcggcgaccccatctacctcggcatccagaaccccgagatgtgcctctactgcgagaaggtcggcgagcagcccactctgcagctcaaggagcagaagatcatggacctctacggccagcccgagcccgtcaagcccttcctcttctaccgcgccaagaccggccgcacctccaccctcgagtccgtcgccttccccgactggttcatcgcctcctccaagcgcgaccagcctattatcctcacctccgagctcggcaagtcctacaacaccgccttcgagctcaacatcaatgac

SEQ ID NO: 99 - DNA, 516 bp, Artificial Sequence
  Synthetic: Codon optimized hIGKV4-hIL-36g
atggtgctccagacccaggtgttcattagcctattactttggatatccggcgcttacggcagcatgtgcaagcctatcaccggcaccatcaacgacctcaaccagcaggtttggacactccagggccagaaccttgtggccgtgcctagatccgactctgttacccctgttacagtggctgtgatcacttgcaagtacccggaagccctggagcagggcaggggagatcctatctatctgggtatccagaacccagaaatgtgcctttattgcgagaaggtgggcgagcagcctacacttcagctgaaggaacagaagatcatggacctctacggacagccagaaccagtgaagcctttcctgttctaccgagccaagaccggccggaccagcaccctggagagcgtggcgttccctgattggttcatcgcctctagcaagagggaccaacctatcatcttaaccagtgagctgggcaagagctacaacacggccttcgagctcaacattaatgat

SEQ ID NO: 100 - DNA, 516 bp, Artificial Sequence
  Synthetic: Codon optimized hIGKV4-hIL-36g
atggtgctccagacccaggtgttcatcagcctattgctctggatcagcggcgcctacggcagcatgtgcaagcccatcaccggcaccatcaacgacttgaaccagcaggtgtggaccttgcagggccagaacctcgtggccgtgccccggagcgacagcgtgacgccagtgaccgtggcggtcatcacctgcaagtaccccgaggccctggagcagggccggggcgaccccatctacctgggcatccagaaccccgagatgtgcctgtactgcgagaaggtgggcgagcagcccacccttcagctgaaggagcagaagatcatggacctgtacggccagcccgagcccgtgaagcccttcctgttctaccgggccaagaccggccggaccagcaccctggagagcgtggccttccccgactggttcatcgccagcagcaagcgggaccagcctatcatcctgaccagcgagctgggcaagagctacaacaccgccttcgagctgaatatcaatgac

SEQ ID NO: 101 - DNA, 516 bp, Artificial Sequence
  Synthetic: Codon optimized hIGKV4-hIL-36g
atggtgctccagacacaggtgttcatctctctcctcctctggatatccggagcctacggctcaatgtgtaagcctatcaccggcactatcaacgatttaaatcagcaggtgtggacccttcagggccagaacctcgtggcagtgccgagaagcgacagcgtgaccccggtgaccgtggccgtgatcacttgtaagtacccagaggccctggagcagggtcgcggcgacccaatctatctgggtattcagaaccctgagatgtgcctgtattgcgagaaggtgggcgaacagccgacgctgcagctcaaggagcagaagatcatggatttatacggccagcctgagccggtgaagccattcctgttctacagggccaagacgggcaggacttccaccttggagagcgtggctttcccggactggttcattgcatcttccaagagggaccagcctattatcctgacaagcgagctgggcaagtcatacaacaccgccttcgagctgaacattaatgac

SEQ ID NO: 102 - DNA, 516 bp, Artificial Sequence
  Synthetic: Codon optimized hIGKV4-hIL-36g
atggtgctccagacccaggtgttcatcagcttgctcctctggatcagcggcgcctacggcagcatgtgcaagcccatcaccggcaccatcaacgacttgaaccagcaggtgtggaccttgcagggccagaacctcgtggccgtgccccggagcgacagcgtgactcctgtgaccgtggcggtgatcacctgcaagtaccccgaggccctggagcagggccggggcgaccccatctacctgggcatccagaaccccgagatgtgcctgtactgcgagaaggtgggcgagcagcccaccctccagctgaaggagcagaagatcatggacctgtacggccagcccgagcccgtgaagcccttcctgttctaccgggccaagaccggccggaccagcaccctggagagcgtggccttccccgactggttcatcgccagcagcaagcgggaccagcctatcatcctgaccagcgagctgggcaagagctacaacaccgccttcgagctgaatatcaacgac

SEQ ID NO: 103 - DNA, 516 bp, Artificial Sequence
  Synthetic: Codon optimized hIGKV4-hIL-36g
atggtgcttcagacacaggtcttcattagcctcttattatggatatccggcgcttacggctctatgtgcaagcctattaccggcacaatcaacgatttgaaccagcaagtgtggaccctccagggccagaatttggtggccgtgccgagatccgatagcgtgaccccagtgaccgtggctgtgattacctgtaagtaccctgaagctctggagcagggcaggggcgacccaatttacctcggcatccagaaccctgagatgtgtctgtactgtgagaaggtgggcgagcagccaactttacaactcaaggaacagaagatcatggacctctacggccagccagagccggttaagcctttcctgttctatagagccaagactggcaggaccagtaccctggagtcagtggctttccctgattggttcattgcctccagcaagcgggatcagccaattattctgaccagcgagctgggaaagagctacaacaccgcgttcgagctgaacatcaacgat

SEQ ID NO: 104 - DNA, 516 bp, Artificial Sequence
  Synthetic: Codon optimized hIGKV4-hIL-36g
atggtgctccagacccaggtgttcatcagcttgctcttgtggatcagcggcgcctacggcagcatgtgcaagcccatcaccggcaccatcaacgacctcaaccagcaggtctggaccctccagggccagaacctcgtcgccgtgcctcgctccgactccgtcactccagtcacagtggctgtgatcacctgcaagtaccccgaggccctcgagcagggccgcggcgaccccatctacctcggcatccagaaccccgagatgtgcctctactgcgagaaggtcggcgagcagcccaccttgcagctcaaggagcagaagatcatggacctctacggccagcccgagcccgtcaagcccttcctcttctaccgcgccaagaccggccgcacctccaccctcgagtccgtcgccttccccgactggttcatcgcctcctccaagcgcgaccagcctattatcctcacctccgagctcggcaagtcctacaacaccgccttcgagctcaatatcaacgac

SEQ ID NO: 105 - DNA, 516 bp, Artificial Sequence
  Synthetic: Codon optimized hIGKV4-hIL-36g
atggtcctccagacccaagtcttcatctccttgttgctctggatcagcggggcctacggctctatgtgtaagcccattaccggcaccatcaacgacctcaaccaacaggtctggacccttcagggtcagaacctcgtcgccgtgcccagatccgactccgtgacccctgtcaccgtggccgtgatcacctgcaaatatcccgaggccctggagcaggggcgcggcgaccccatatacctgggcatccagaaccccgagatgtgcctctactgcgagaaggtgggcgaacagcccaccctccagctgaaggagcagaagatcatggacctgtacggccagcccgagcccgtgaagcccttcctgttctatagggccaagaccggccgcacctccaccctggagtccgtggccttccccgattggtttattgccagtagcaagagggaccagcccatcatcctcaccagcgaactgggcaagagctacaacaccgccttcgagctgaacatcaatgac

SEQ ID NO: 106 - DNA, 516 bp, Artificial Sequence
  Synthetic: Codon optimized hIGKV4-hIL-36g
atggtgctccagacacaggtgttcatcagcctcctcctctggatcagcggggcctacggcagcatgtgcaagcccatcacaggcaccatcaacgacctcaatcagcaagtctggaccctccagggtcagaacctcgtggccgtgccccgcagcgacagcgtgacgcccgtgacagtggccgtcatcacgtgcaaataccccgaagccctggagcagggccgtggcgaccctatctacctgggcatacagaaccccgagatgtgcctgtactgcgagaaggtgggtgagcagcccaccctgcaactgaaggagcagaagatcatggacctctacggacaaccggagcccgtgaaacccttcctgttctacagggccaagaccgggaggacctccaccctggaaagcgtggcctttcccgactggtttatcgccagctccaagagggaccaacccatcatcctcaccagcgagctgggcaagtcttacaacaccgcctttgagctgaacatcaatgat

SEQ ID NO: 107 - DNA, 516 bp, Artificial Sequence
  Synthetic: Codon optimized hIGKV4-hIL-36g
atggtgctccagacccaggtgttcatcagcctcctcctctggatcagcggggcctacgggagcatgtgcaagcccatcaccgggaccatcaacgacctcaaccagcaggtctggacgctccaggggcagaatctcgtggccgtgcccagatccgacagcgtgaccccggtgaccgtggccgtcatcacctgtaagtacccggaggccctggaacagggccgaggtgaccccatctatctgggtatccagaatccggagatgtgcctgtactgcgagaaggtgggcgagcagcccaccctgcagctgaaggagcagaagatcatggacctgtacggccaacccgagcccgtgaagcccttcctgttttacagggccaagaccggccggacgagcaccctggagagcgtggcctttcccgactggttcatcgccagtagcaagagggaccaacccatcatcctgacctccgagctgggcaagagctacaataccgccttcgagctcaacatcaatgat

SEQ ID NO: 108 - DNA, 516 bp, Artificial Sequence
  Synthetic: Codon optimized hIGKV4-hIL-36g
atggtcctacagacccaagtgttcatcagcctccttctctggatcagcggagcctacggctccatgtgtaagcccatcaccggcactatcaacgacctcaatcagcaggtgtggacactccagggccagaacctcgtggccgtgcccagaagcgacagcgtgaccccggtcaccgtcgccgtgatcacctgcaaatatcccgaggccctggagcagggccgaggggaccccatctacctcgggatccagaacccggagatgtgtctgtattgtgagaaggtcggcgagcaacctaccctgcagctgaaggagcagaagatcatggacctgtacggccagcccgagccggtgaaaccgttcctgttctaccgggccaagaccggcagaaccagcaccctggaaagcgtggcctttcccgactggttcatcgcgagcagtaaacgggaccaacccatcatcctgaccagcgagctgggcaagagctacaacaccgcgtttgagctgaacatcaacgac

SEQ ID NO: 109 - DNA, 516 bp, Artificial Sequence
  Synthetic: Codon optimized hIGKV4-hIL-36g
atggtgctacagacccaggtgttcatcagcctcctactttggatcagcggggcgtacggcagcatgtgcaaacccatcacaggaaccatcaacgaccttaaccagcaggtctggacactccagggccagaacctcgtggccgtgcccaggagcgattccgtcacgcccgtgaccgtggctgtgatcacctgcaagtaccccgaggccctggagcaggggcgaggggaccccatctacctgggcatccagaaccccgagatgtgcctgtactgcgagaaggtcggtgaacagcccaccctccaactcaaggagcagaagattatggacctgtacggccagccagagcccgtgaagccatttctgttctatagggccaagaccggccgcacctccaccctggagtccgtggccttccccgactggttcatcgccagcagcaaacgggaccagcccatcattctgaccagcgaactgggcaagagctacaataccgccttcgagcttaatatcaatgac

SEQ ID NO: 110 - DNA, 516 bp, Artificial Sequence
  Synthetic: Codon optimized hIGKV4-hIL-36g
atggtgctccaaactcaggtgttcatcagcctcctcctctggatcagcggggcgtacggcagcatgtgtaagcccatcaccggcaccatcaacgacctcaaccagcaagtgtggaccttgcagggccagaatctcgtggccgtgcccaggtccgacagcgtgacgcccgtgactgtggccgtcatcacctgcaaatatccggaggcgctggagcagggcagaggcgatcccatctatctcgggatccagaaccccgagatgtgcctgtattgcgagaaggtcggcgagcagcccaccctccagctgaaggagcagaagatcatggacctgtatggccagcccgagcccgtgaagcccttcctgttctaccgggcgaagaccggccgcacctccaccctggaaagcgtggccttccccgattggttcatcgcgtccagcaagagggaccagccgatcatcctgacctcagagctgggcaagtcctacaacaccgccttcgagctgaatatcaacgac

SEQ ID NO: 111 - DNA, 516 bp, Artificial Sequence
  Synthetic: Codon optimized hIGKV4-hIL-36g
atggtgctccagacccaggtgttcataagcctcctcctctggatcagcggcgcctacggctctatgtgcaagcccatcaccgggaccatcaacgacctcaaccagcaggtgtggaccctacagggccagaacctcgtggccgtgccccggagcgactctgtgactcccgtcaccgtggccgtcatcacctgcaagtaccccgaggccctggagcagggcaggggcgacccgatctatctgggcatccagaatcccgagatgtgcctctactgcgagaaggtgggcgaacagcccaccctccagctgaaggagcagaagataatggatctgtacggtcagcccgagcccgtgaagccgttcctgttctaccgggccaagacgggaaggacaagcaccctggagagcgtggcatttcccgactggttcatcgccagctccaagagggatcagcccataatcctgaccagcgagctgggcaagagctacaacaccgccttcgagctgaatatcaacgac

SEQ ID NO: 112 - DNA, 516 bp, Artificial Sequence
  Synthetic: Codon optimized hIGKV4-hIL-36g
atggtgctccagacccaagtcttcatcagcctcctcctctggatctccggcgcctacgggagcatgtgcaagcccatcacgggcaccatcaacgacctcaatcagcaggtctggaccctccagggtcagaacctcgtggccgtccccaggtccgacagcgtgaccccggtgaccgtggccgtgatcacctgcaagtaccccgaggcgctggagcaaggccggggcgaccccatctacctgggtatccagaaccccgagatgtgcctgtactgtgagaaagtgggcgagcagcccacactgcagctgaaggagcagaagatcatggatctgtacggtcagcccgagcccgtgaaacccttcctgttttacagggccaagaccggcaggaccagcaccctggagagcgtggccttcccggactggttcatcgccagcagtaagagggaccaacccataatactgaccagcgagctcggcaagagctacaataccgccttcgagctgaatatcaacgac

SEQ ID NO: 113 - DNA, 516 bp, Artificial Sequence
  Synthetic: Codon optimized hIGKV4-hIL-36g
atggtgttgcagacacaggtgttcatcagcctcctcctctggatcagcggcgcttacggcagcatgtgcaagcccatcaccggcaccatcaacgatctcaatcagcaggtgtggaccctccagggccagaatctcgtagccgttcccagaagcgacagcgtgacgcccgtcacggtggctgtgatcacgtgcaaatacccagaggcactcgagcagggcagaggcgatcctatctacctgggaatccagaaccccgagatgtgcctgtactgcgagaaggtcggagagcagcctaccctgcaactgaaggagcagaagataatggacctgtacggacagcccgagcccgtgaagccatttctgttctacagagccaagaccggaagaacaagcacactggaaagcgtggcatttcctgactggttcattgccagctccaagcgggaccagcccataatcctcacctctgagctgggcaagagctacaacaccgccttcgagctgaacatcaacgac

SEQ ID NO: 114 - DNA, 516 bp, Artificial Sequence
  Synthetic: Codon optimized hIGKV4-hIL-36g
atggtgctccagacacaggtgttcatcagcctcctcctctggatcagtggcgcgtacggatcaatgtgcaagcccatcacaggcaccattaacgatctcaaccagcaggtgtggaccctccagggccagaacctcgtggccgtgcccaggtccgacagcgtgactcctgtcacagtagccgtgatcacctgcaagtaccccgaggcacttgagcagggccggggcgaccccatctacctggggatccagaaccctgagatgtgtctgtactgcgagaaagtgggcgagcagcccacactgcagctcaaggagcagaagatcatggatctgtatggccagcccgagcccgtgaagcctttcctgttttatcgcgccaagacaggacggacttcaaccttggaatccgtggctttccccgactggttcatcgcgtcttccaagagggaccagcctatcattcttacctcagagctgggcaaatcatataacacagctttcgagctgaacatcaatgac

SEQ ID NO: 115 - DNA, 516 bp, Artificial Sequence
  Synthetic: Codon optimized murine mIL-2-mIL-36g
atgtacagcatgcagctcgcatcctgtgtcacattgacacttgtgctccttgtcaacagcggaagagaaactcctgactttggggaggtttttgacttggaccagcaggtgtggatctttcgtaatcaggcccttgtgacagttccacgaagccacagagtaaccccagtcagcgtgactatcctcccatgcaagtacccagagtctcttgaacaggacaaagggattgccatttatttgggaattcagaatccagataaatgcctgttttgtaaggaagttaatggacaccctactttgctgctaaaggaagagaagattttggatttgtaccaccaccctgagccaatgaagccattcctgttttaccacacccggacaggtggaacatccacctttgaatcagtggctttccctggccactatattgcctcctccaagactggcaaccccatcttcctcacatcaaagaagggagaatattacaacattaacttcaatttagatataaagtct

SEQ ID NO: 116 - DNA, 549 bp, Artificial Sequence
  Synthetic: Codon optimized human OX40L
atggaaagggtccaacccctggaagagaatgtgggaaatgcagccaggccaagattcgagaggaacaagctattgctggtggcctctgtaattcagggactggggctgctcctgtgcttcacctacatctgcctgcacttctctgctcttcaggtatcacatcggtatcctcgaattcaaagtatcaaagtacaatttaccgaatataagaaggagaaaggtttcatcctcacttcccaaaaggaggatgaaatcatgaaggtgcagaacaactcagtcatcatcaactgtgatgggttttatctcatctccctgaagggctacttctcccaggaagtcaacattagccttcattaccagaaggatgaggagcccctcttccaactgaagaaggtcaggtctgtcaactccttgatggtggcctctctgacttacaaagacaaagtctacttgaatgtgaccactgacaatacctccctggatgacttccatgtgaatggcggagaactgattcttatccatcaaaatcctggtgaattctgtgtcctt

SEQ ID NO: 117 - DNA, 594 bp, Artificial Sequence
  Synthetic: Codon optimized mouse OX40L
atggaaggggaaggggttcaacccctggatgagaatctggaaaacggatcaaggccaagattcaagtggaagaagacgctaaggctggtggtctctgggatcaagggagcagggatgcttctgtgcttcatctatgtctgcctgcaactctcttcctctccggcaaaggaccctccaatccaaagactcagaggagcagttaccagatgtgaggatgggcaactattcatcagctcatacaagaatgagtatcaaactatggaggtgcagaacaattcggttgtcatcaagtgcgatgggctttatatcatctacctgaagggctcctttttccaggaggtcaagattgaccttcatttccgggaggatcataatcccatctctattccaatgctgaacgatggtcgaaggattgtcttcactgtggtggcctctttggctttcaaagataaagtttacctgactgtaaatgctcctgatactctctgcgaacacctccagataaatgatggggagctgattgttgtccagctaacgcctggatactgtgctcctgaaggatcttaccacagcactgtgaaccaagtaccactg

SEQ ID NO: 118 - RNA, 92 nt, Artificial Sequence
  Synthetic: 5UTR-019
ucaagcuuuuggacccucguacagaagcuaauacgacucacuauagggaaauaagagagaaaagaagaguaagaagaaauauaagagccacc

SEQ ID NO: 119 - RNA, 118 nt, Artificial Sequence
  Synthetic: 3UTR-019
ugauaauaggcuggagccucgguggccaugcuucuugccccuugggccuccccccagccccuccuccccuuccugcacccguacccccuggucuuugaauaaagucugagugggcggc

SEQ ID NO: 120 - RNA, 141 nt, Artificial Sequence
  Synthetic: 3UTR-019 + miR-122 binding site
ugauaauaggcuggagccucgguggccaugcuucuugccccuugggccuccccccagccccuccuccccuuccugcacccguaccccccaaacaccauugucacacuccaguggucuuugaauaaagucugagugggcggc

SEQ ID NO: 121 - RNA, 549 nt, Artificial Sequence
  Synthetic: Codon-optimized sequence 1 for ENSP 281834
auggagagagugcagccccuggaggagaacgugggcaacgccgccagacccagauucgagagaaacaagcugcugcugguggccagcgugauccagggccugggccugcugcugugcuucaccuacaucugccugcacuucagcgcccugcaggugagccacagauaccccagaauccagagcaucaaggugcaguucaccgaguacaagaaggagaagggcuucauccugaccagccagaaggaggacgagaucaugaaggugcagaacaacagcgugaucaucaacugcgacggcuucuaccugaucagccugaagggcuacuucagccaggaggugaacaucagccugcacuaccagaaggacgaggagccccuguuccagcugaagaaggugagaagcgugaacagccugaugguggccagccugaccuacaaggacaagguguaccugaacgugaccaccgacaacaccagccuggacgacuuccacgugaacggcggcgagcugauccugauccaccagaaccccggcgaguucugcgugcug

SEQ ID NO: 122 - RNA, 549 nt, Artificial Sequence
  Synthetic: Codon-optimized sequence 2 for ENSP 281834
auggagcgugugcagccucuugaggagaaugugggaaaugcagcccggccucgauucgaacguaauaaacuccugcucguggccuccgugauccagggucucgguuuauugcuguguuuuaccuauauaugcuuacacuuuagugcauuacaggucucacaccgguacccucgcauucagucuauaaaagugcaguuuaccgaguauaagaaggagaaagguuuuauacugacuucucagaaagaggacgagaucaugaaggugcagaauaauagcgucauuaucaacugcgauggauucuaucuaauuucccuaaagggguacuucagccaggaggucaauauaucacugcacuaucaaaaggacgaggagccccuguuucaacugaagaaagugcgaucaguuaacucucugaugguugccucucugaccuauaaggacaaagucuacuugaacgugacaacugacaacaccucacuggaugacuuucaugugaaugggggggaacugauucuuauccaucagaauccaggagaauucugugugcuc

SEQ ID NO: 123 - RNA, 549 nt, Artificial Sequence
  Synthetic: Codon-optimized sequence 3 for ENSP 281834
auggagcgggugcagccccuggaggagaaugugggcaaugcugcccggcccagguuugaaagaaacaagcugcugcugguggccagcgucauccagggccugggccugcugcugugcuucaccuacaucugccugcacuucagcgcccugcaggugagccaccgcuacccccgcauccagagcaucaaggugcaguucacagaguacaagaaggagaagggcuucauccugaccagccagaaggaggaugagaucaugaaggugcagaacaacagcgucaucaucaacugugauggcuucuaccugaucagccugaagggcuacuucagccaggaggugaacaucagccugcacuaccagaaggaugaggagccccucuuccagcugaagaaggugcgcucugugaacagccugaugguggccagccugaccuacaaggacaagguguaccugaaugugaccacagacaacaccagccuggaugacuuccacgugaauggaggagagcugauccugauccaccagaacccuggagaguucugugugcug

SEQ ID NO: 124 - RNA, 549 nt, Artificial Sequence
  Synthetic: Codon-optimized sequence 4 for ENSP 281834
auggagcgggugcagccccuggaggagaacgugggcaacgccgcccgcccgcguuuugagcgaaauaaguuacugcuuguugcaucugugauacagggguuggguuuacuucuuugcuuuacauauauuugucuccacuuuagugcgcuucagguaucccaucgguacccgcgcauccagucaaucaagguccaguucacugaauauaaaaaggagaaaggauucauucugacuucacaaaaagaggacgaaaucaugaaagugcagaacaacucuguaauuauaaacugcgauggguucuaucugaucagucugaagggauauuuuagccaggaaguaaauauuucacuacauuaucagaaggacgaagaaccacuuuuucaacugaagaaaguccgguccgugaacucccugaugguugcuagccuuaccuacaaggauaaagucuauuuaaacgucacaacagauaacacuagccucgacgauuuccaugugaacggaggugaacugauauugauccaucaaaaccccggcgaguucugcguuuua

SEQ ID NO: 125 - RNA, 549 nt, Artificial Sequence
  Synthetic: Codon-optimized sequence 5 for ENSP 281834
auggagcggguccagccccucgaggagaacguugguaaugccgcacgucccagguuugaacgcaacaagcugcuguugguggccagcgucauucaggggcuggguuuguugcugugcuucacuuacaucugucugcauuuuagugcacuccaggugucccaccgcuacccccguauccaauccauuaaaguccaauuuaccgaauacaaaaaagagaaggguuucauucuuaccucccagaaggaggaugaaauuaugaaggugcagaacaauucuguuaucaucaacugugacggauucuaucugauuucacugaagggauacuuuucccaggaggugaacaucagucugcauuaucagaaggacgaagaaccgcuuuuucaacugaagaagguuaggagugugaacuccuuaaugguagccagccugacauauaaggacaagguauaucugaacgucaccacugauaacaccucuuuagacgauuuucauguaaaugggggagaauugauacucauucaccagaauccgggugaguuuuguguucug

SEQ ID NO: 126 - RNA, 399 nt, Artificial Sequence
  Synthetic: Codon-optimized sequence 1 for ENSP 356691
auggugagccacagauaccccagaauccagagcaucaaggugcaguucaccgaguacaagaaggagaagggcuucauccugaccagccagaaggaggacgagaucaugaaggugcagaacaacagcgugaucaucaacugcgacggcuucuaccugaucagccugaagggcuacuucagccaggaggugaacaucagccugcacuaccagaaggacgaggagccccuguuccagcugaagaaggugagaagcgugaacagccugaugguggccagccugaccuacaaggacaagguguaccugaacgugaccaccgacaacaccagccuggacgacuuccacgugaacggcggcgagcugauccugauccaccagaaccccggcgaguucugcgugcug

SEQ ID NO: 127 - RNA, 399 nt, Artificial Sequence
  Synthetic: Codon-optimized sequence 2 for ENSP 356691
augguuucucaccguuacccacggauccagucuaucaagguucaguuuaccgaguacaaaaaggaaaaaggguucauccucaccucucagaaagaggacgaaaucaugaaggugcagaauaacucuguaaucauuaauugcgacgguuuuuaucugauuucacugaagggcuacuuuagucaggaaguuaauauuaguuugcacuaccaaaaggacgaggagccucucuuccaacuaaaaaagguaagauccguuaauucccuuaugguggccuccuuaacuuauaaggacaagguguaucugaaugugaccacagauaacacaucccuggacgacuuucauguaaauggcggcgaguuaauucugauacaccagaacccuggcgaguucugcgugcug

SEQ ID NO: 128 - RNA, 399 nt, Artificial Sequence
  Synthetic: Codon-optimized sequence 3 for ENSP 356691
auggugagccaccgcuacccccgcauccagagcaucaaggugcaguucacagaguacaagaaggagaagggcuucauccugaccagccagaaggaggaugagaucaugaaggugcagaacaacagcgucaucaucaacugugauggcuucuaccugaucagccugaagggcuacuucagccaggaggugaacaucagccugcacuaccagaaggaugaggagccccucuuccagcugaagaaggugcgcucugugaacagccugaugguggccagccugaccuacaaggacaagguguaccugaaugugaccacagacaacaccagccuggaugacuuccacgugaauggaggagagcugauccugauccaccagaacccuggagaguucugugugcug

SEQ ID NO: 129 - RNA, 399 nt, Artificial Sequence
  Synthetic: Codon-optimized sequence 4 for ENSP 356691
auggugagccaccgguacccccggauccagagcaucaaggugcaguucaccgaauacaagaaggagaaggguuuuauccugacgagccagaaggaagacgagauuaugaagguccaaaacaacucagucaucauaaacugcgauggauuuuaccugaucucucugaaaggguacuucucccaggaagugaauauuagcuugcacuaucaaaaagaugaggagccucuauuccagcucaagaaggucagaagcgucaauagucugauggucgcaucauuaaccuauaaagacaaaguauaucuaaaugugacgacagacaauacaucccucgaugauuuucacgucaacggaggcgaacucauucugauccaccagaauccaggggaauuuugcgugcug

SEQ ID NO: 130 - RNA, 399 nt, Artificial Sequence
  Synthetic: Codon-optimized sequence 5 for ENSP 356691
auggucucacaccgguacccccguauccagaguauuaaggugcaauucacggaguauaaaaaagaaaagggauucauucugacgucucagaaggaagaugagaucaugaagguccagaacaauucugugaucauuaauugcgauggauuuuaucugauuucacuuaaaggauauuuuucccaggagguuaauaucaguuugcacuaucagaaagacgaggagccauuauuccagcugaagaaggugagaucagugaauagccugaugguugcgucacugacguauaaagacaaaguuuaucuaaacguuaccacugauaauacaucccuugaugauuuucaugugaacgggggugaacugauccuuauacaccagaaccccggagaguucuguguguug

SEQ ID NO: 131 - RNA, 399 nt, Artificial Sequence; identical to SEQ ID NO: 126
  Synthetic: Codon-optimized sequence 1 for ENSP 439704

SEQ ID NO: 132 - RNA, 399 nt, Artificial Sequence
  Synthetic: Codon-optimized sequence 2 for ENSP 439704
auggugucacaccgguacccucggauccagucuauuaaaguucaauuuacggaguacaagaaagaaaaaggcuuuauccuuacaagccaaaaggaagacgagaucaugaaagugcaaaacaacagugugauuauaaauugugauggcuucuaccuuauuagucugaagggcuacuuuagucaggaagucaauauuagccuacacuaccagaaagacgaggagccccucuuucaacugaaaaaggugcgcuccgugaauucguugauggucgccucucugaccuacaaagauaagguguaucuuaacguuacuaccgacaauacuagucuggacgacuuucacgucaacggaggcgaacuuauucugauccaccagaaccccggcgaauucugcgugcug

SEQ ID NO: 133 - RNA, 399 nt, Artificial Sequence; identical to SEQ ID NO: 128
  Synthetic: Codon-optimized sequence 3 for ENSP 439704

SEQ ID NO: 134 - RNA, 399 nt, Artificial Sequence
  Synthetic: Codon-optimized sequence 4 for ENSP 439704
auggugagccaccgguacccccggauccagagcaucaaggugcaguucacagaguacaagaaggagaagggauuuauucucacaagucagaaagaagaugagaucaugaagguucagaacaacucagucauuauuaauugcgacggauucuaucucauuagccucaaaggcuauuucagccaggaggucaauaucagccugcacuaccagaaggaugaggaaccucucuuucagcugaaaaaaguccgcucugugaauucccucauggucgcuucccugaccuacaaggauaaaguuuauuugaacguuacaacagauaauacaucgcuggacgacuuccaugugaaugguggcgaacuaauucuaauacaccaaaauccaggcgaauuuuguguccuu

SEQ ID NO: 135 - RNA, 399 nt, Artificial Sequence
  Synthetic: Codon-optimized sequence 5 for ENSP 439704
augguaucccauagauacccacguauucaaagcauuaaggugcaguucacagaguacaaaaaggagaaggguuucauacugacgucacagaaggaggacgagauaaugaaggugcagaauaauagugugaucaucaauugugauggauucuauuugaucagccucaaagguuauuucucacaggaagucaacauuucccugcacuaccagaaggacgaagagccuuuguuucagcugaagaaggugcgcucagugaacaguuugaugguagccucccuaacuuauaaagauaaaguuuaucugaacgugacaaccgauaacacaucccuggacgacuuucacgucaauggaggugaguuaauccugauccaucagaaucccggagaauucugcguucuu

SEQ ID NO: 136 - protein, 5 aa, Artificial Sequence
  Synthetic: linker
GGGGS

SEQ ID NO: 137 - protein, 6 aa, Artificial Sequence
  Synthetic: linker
GGGGGS

SEQ ID NO: 138 - protein, 7 aa, Artificial Sequence
  Synthetic: linker
GGGGGGS

SEQ ID NO: 139 - protein, 8 aa, Artificial Sequence
  Synthetic: linker
GGGGGGGS

SEQ ID NO: 140 - protein, 505 aa, Homo sapiens
  Amino Acid sequence of human IL-23 (IL-12p40 subunit and IL-23p19 subunit linked by GS Linker)
MCHQQLVISWFSLVFLASPLVAIWELKKDVYVVELDWYPDAPGEMVVLTCDTPEEDGITWTLDQSSEVLGSGKTLTIQVKEFGDAGQYTCHKGGEVLSHSLLLLHKKEDGIWSTDILKDQKEPKNKTFLRCEAKNYSGRFTCWWLTTISTDLTFSVKSSRGSSDPQGVTCGAATLSAERVRGDNKEYEYSVECQEDSACPAAEESLPIEVMVDAVHKLKYENYTSSFFIRDIIKPDPPKNLQLKPLKNSRQVEVSWEYPDTWSTPHSYFSLTFCVQVQGKSKREKKDRVFTDKTSATVICRKNASISVRAQDRYYSSSWSEWASVPCSGGGGGGSRAVPGGSSPAWTQCQQLSQKLCTLAWSAHPLVGHMDLREEGDEETTNDVPHIQCGDGCDPQGLRDNSQFCLQRIHQGLIFYEKLLGSDIFTGEPSLLPDSPVGQLHASLLGLSQLLQPEGHHWETQQIPSLSPSQPWQRLLLRFKILRSLQAFVAVAARVFAHGAATLSP

SEQ ID NO: 141 - RNA, 1515 nt, Homo sapiens
  Nucleotide sequence (ORF) of human IL-23 (IL-12p40 subunit and IL-23p19 subunit linked by GS Linker)
augugucaccagcaguuggucaucucuugguuuucccugguauuucuggcaucuccccucguggccauaugggaacugaagaaagauguuuaugucguagaauuggauugguauccggaugccccuggagaaauggugguccucaccugugacaccccugaagaagaugguaucaccuggaccuuggaccagagcagugaggucuuaggcucuggcaagacccugaccauccaagucaaagaguuuggagaugcuggccaguacaccugucacaaaggaggcgagguucuaagccauucgcuccugcugcuucacaagaaggaagauggaauuugguccacugauauuuuaaaggaccagaaagaacccaagaauaagaccuuucuaagaugcgaggccaagaauuauucuggacguuucaccugcugguggcugacgacaaucaguacugauuugacauucagugucaagagcagcagaggcucuucugacccccaaggggugacgugcggagcugcuacacucucugcagagagagucagaggggacaacaaggaguaugaguacucaguggagugccaggaggacagugccugcccagcugcugaggagagucugcccauugaggucaugguggaugccguucacaagcucaaguaugagaacuacaccagcagcuucuucaucagggacaucaucaaaccugacccacccaagaacuugcagcugaagccauuaaagaauucucggcagguggaggucagcugggaguacccugacaccuggaguacuccacauuccuacuucucccugacauucugcguucagguccagggcaagagcaagagagagaagaaagauagagucuucacggacaagaccucagccacggucaucugccgcaagaaugccagcauuagcgugcgggcccaggaccgcuacuauagcucaucuuggagcgaaugggcaucugugcccugcaguggcggagggggcggagggagcagagcugugccugggggcagcagcccugccuggacucagugccagcagcuuucacagaagcucugcacacuggccuggagugcacauccacuagugggacacauggaucuaagagaagagggagaugaagagacuacaaaugauguuccccauauccaguguggagauggcugugacccccaaggacucagggacaacagucaguucugcuugcaaaggauccaccagggucugaucuuuuaugagaagcugcuaggaucggauauuuucacaggggagccuucucugcucccugauagcccugugggccagcuucaugccucccuacugggccucagccaacuccugcagccugagggucaccacugggagacucagcagauuccaagccucagucccagccagccauggcagcgucuccuucuccgcuucaagauccuucgcagccuccaggccuuuguggcuguagccgcccgggucuuugcccauggagcagcaacccugaguccc

SEQ ID NO: 142 - RNA, 1807 nt, Homo sapiens
  Full-length mRNA Nucleotide sequence (5 UTR, ORF, 3 UTR, mir-122-5p polyA tail) of human IL-23 (IL-12p40 subunit and IL-23p19 subunit linked by GS Linker)
  misc_feature 1..1: /note="7MeGpppG2'OMe at 5' end"
  misc_feature 1..1807: /note="Every A,C G and U = AMP, CMP, GMP and N1-psi -UMP, respectively"
ggaaauaagagagaaaagaagaguaagaagaaauauaagagccaccaugugucaccagcaguuggucaucucuugguuuucccugguauuucuggcaucuccccucguggccauaugggaacugaagaaagauguuuaugucguagaauuggauugguauccggaugccccuggagaaauggugguccucaccugugacaccccugaagaagaugguaucaccuggaccuuggaccagagcagugaggucuuaggcucuggcaagacccugaccauccaagucaaagaguuuggagaugcuggccaguacaccugucacaaaggaggcgagguucuaagccauucgcuccugcugcuucacaagaaggaagauggaauuugguccacugauauuuuaaaggaccagaaagaacccaagaauaagaccuuucuaagaugcgaggccaagaauuauucuggacguuucaccugcugguggcugacgacaaucaguacugauuugacauucagugucaagagcagcagaggcucuucugacccccaaggggugacgugcggagcugcuacacucucugcagagagagucagaggggacaacaaggaguaugaguacucaguggagugccaggaggacagugccugcccagcugcugaggagagucugcccauugaggucaugguggaugccguucacaagcucaaguaugagaacuacaccagcagcuucuucaucagggacaucaucaaaccugacccacccaagaacuugcagcugaagccauuaaagaauucucggcagguggaggucagcugggaguacccugacaccuggaguacuccacauuccuacuucucccugacauucugcguucagguccagggcaagagcaagagagagaagaaagauagagucuucacggacaagaccucagccacggucaucugccgcaagaaugccagcauuagcgugcgggcccaggaccgcuacuauagcucaucuuggagcgaaugggcaucugugcccugcaguggcggagggggcggagggagcagagcugugccugggggcagcagcccugccuggacucagugccagcagcuuucacagaagcucugcacacuggccuggagugcacauccacuagugggacacauggaucuaagagaagagggagaugaagagacuacaaaugauguuccccauauccaguguggagauggcugugacccccaaggacucagggacaacagucaguucugcuugcaaaggauccaccagggucugaucuuuuaugagaagcugcuaggaucggauauuuucacaggggagccuucucugcucccugauagcccugugggccagcuucaugccucccuacugggccucagccaacuccugcagccugagggucaccacugggagacucagcagauuccaagccucagucccagccagccauggcagcgucuccuucuccgcuucaagauccuucgcagccuccaggccuuuguggcuguagccgcccgggucuuugcccauggagcagcaacccugagucccugauaauaggcuggagccucgguggccaugcuucuugccccuugggccuccccccagccccuccuccccuuccugcacccguaccccccaaacaccauugucacacuccaguggucuuugaauaaagucugagugggcggcaaaaaaaaaaaaaaaaaaaaaaaaaaaaaaaaaaaaaaaaaaaaaaaaaaaaaaaaaaaaaaaaaaaaaaaaaaaaaaaaaaaaaaaaaaaaaaaaaaaaucuag

SEQ ID NO: 143 - RNA, 516 nt, Homo sapiens
  Human IL-36-gamma mRNA (ORF)
augguguugcagacccaggucuucauuucucuguugcucuggaucucuggugccuacgggucaauguguaaaccuauuacugggacuauuaaugauuugaaucagcaaguguggacccuucagggucagaaccuuguggcaguuccacgaagugacagugugaccccagucacuguugcuguuaucacaugcaaguauccagaggcucuugagcaaggcagaggggaucccauuuauuugggaauccagaauccagaaauguguuuguauugugagaagguuggagaacagcccacauugcagcuaaaagagcagaagaucauggaucuguauggccaacccgagcccgugaaacccuuccuuuucuaccgugccaagacugguaggaccuccacccuugagucuguggccuucccggacugguucauugccuccuccaagagagaccagcccaucauucugacuucagaacuugggaagucauacaacacugccuuugaauuaaauauaaaugac

SEQ ID NO: 144 - RNA, 808 nt, Homo sapiens
  Full-length mRNA Nucleotide sequence (5 UTR, ORF, 3 UTR, mir-122-5p polyA tail) of human IL-36-gamma
  misc_feature 1..1: /note="7MeGpppG2'OMe at 5' end"
  misc_feature 1..808: /note="Every A,C G and U = AMP, CMP, GMP and N1-psi -UMP, respectively"
ggaaauaagagagaaaagaagaguaagaagaaauauaagagccaccaugguguugcagacccaggucuucauuucucuguugcucuggaucucuggugccuacgggucaauguguaaaccuauuacugggacuauuaaugauuugaaucagcaaguguggacccuucagggucagaaccuuguggcaguuccacgaagugacagugugaccccagucacuguugcuguuaucacaugcaaguauccagaggcucuugagcaaggcagaggggaucccauuuauuugggaauccagaauccagaaauguguuuguauugugagaagguuggagaacagcccacauugcagcuaaaagagcagaagaucauggaucuguauggccaacccgagcccgugaaacccuuccuuuucuaccgugccaagacugguaggaccuccacccuugagucuguggccuucccggacugguucauugccuccuccaagagagaccagcccaucauucugacuucagaacuugggaagucauacaacacugccuuugaauuaaauauaaaugacugauaauaggcuggagccucgguggccaugcuucuugccccuugggccuccccccagccccuccuccccuuccugcacccguaccccccaaacaccauugucacacuccaguggucuuugaauaaagucugagugggcggcaaaaaaaaaaaaaaaaaaaaaaaaaaaaaaaaaaaaaaaaaaaaaaaaaaaaaaaaaaaaaaaaaaaaaaaaaaaaaaaaaaaaaaaaaaaaaaaaaaaaucuag

SEQ ID NO: 145 - RNA, 549 nt, Homo sapiens; identical to SEQ ID NO: 66
  Human OX40L mRNA (ORF)

SEQ ID NO: 146 - RNA, 841 nt, Homo sapiens
  Full-length mRNA Nucleotide sequence (5 UTR, ORF, 3 UTR, miR-122-5p polyA tail) of human OX40L
  misc_feature 1..1: /note="7MeGpppG2'OMe at 5' end"
  misc_feature 1..841: /note="Every A,C G and U = AMP, CMP, GMP and N1-psi -UMP, respectively"
ggaaauaagagagaaaagaagaguaagaagaaauauaagagccaccauggaaaggguccaaccccuggaagagaaugugggaaaugcagccaggccaagauucgagaggaacaagcuauugcugguggccucuguaauucagggacuggggcugcuccugugcuucaccuacaucugccugcacuucucugcucuucagguaucacaucgguauccucgaauucaaaguaucaaaguacaauuuaccgaauauaagaaggagaaagguuucauccucacuucccaaaaggaggaugaaaucaugaaggugcagaacaacucagucaucaucaacugugauggguuuuaucucaucucccugaagggcuacuucucccaggaagucaacauuagccuucauuaccagaaggaugaggagccccucuuccaacugaagaaggucaggucugucaacuccuugaugguggccucucugacuuacaaagacaaagucuacuugaaugugaccacugacaauaccucccuggaugacuuccaugugaauggcggagaacugauucuuauccaucaaaauccuggugaauucuguguccuuugauaauaggcuggagccucgguggccaugcuucuugccccuugggccuccccccagccccuccuccccuuccugcacccguaccccccaaacaccauugucacacuccaguggucuuugaauaaagucugagugggcggcaaaaaaaaaaaaaaaaaaaaaaaaaaaaaaaaaaaaaaaaaaaaaaaaaaaaaaaaaaaaaaaaaaaaaaaaaaaaaaaaaaaaaaaaaaaaaaaaaaaaucuag

SEQ ID NO: 147 - protein, 193 aa, Homo sapiens
  Human IL 18 isoform 1
MAAEPVEDNCINFVAMKFIDNTLYFIAEDDENLESDYFGKLESKLSVIRNLNDQVLFIDQGNRPLFEDMTDSDCRDNAPRTIFIISMYKDSQPRGMAVTISVKCEKISTLSCENKIISFKEMNPPDNIKDTKSDIIFFQRSVPGHDNKMQFESSSYEGYFLACEKERDLFKLILKKEDELGDRSIMFTVQNED

SEQ ID NO: 148 - DNA, 579 bp, Homo sapiens
  Nucleotide sequence of IL-18 isoform 1 (Precursor)
atggctgctgaaccagtagaagacaattgcatcaactttgtggcaatgaaatttattgacaatacgctttactttatagctgaagatgatgaaaacctggaatcagattactttggcaagcttgaatctaaattatcagtcataagaaatttgaatgaccaagttctcttcattgaccaaggaaatcggcctctatttgaagatatgactgattctgactgtagagataatgcaccccggaccatatttattataagtatgtataaagatagccagcctagaggtatggctgtaactatctctgtgaagtgtgagaaaatttcaactctctcctgtgagaacaaaattatttcctttaaggaaatgaatcctcctgataacatcaaggatacaaaaagtgacatcatattctttcagagaagtgtcccaggacatgataataagatgcaatttgaatcttcatcatacgaaggatactttctagcttgtgaaaaagagagagacctttttaaactcattttgaaaaaagaggatgaattgggggatagatctataatgttcactgttcaaaacgaagac

SEQ ID NO: 149 - protein, 157 aa, Homo sapiens
  Amino acid sequence of IL-18 isoform 1 (Mature)
YFGKLESKLSVIRNLNDQVLFIDQGNRPLFEDMTDSDCRDNAPRTIFIISMYKDSQPRGMAVTISVKCEKISTLSCENKIISFKEMNPPDNIKDTKSDIIFFQRSVPGHDNKMQFESSSYEGYFLACEKERDLFKLILKKEDELGDRSIMFTVQNED

SEQ ID NO: 150 - skipped

SEQ ID NO: 151 - protein, 189 aa, Homo sapiens
  Amino acid sequence of isoform 2, Delta3pro-IL-18, 27-30 missing (Precursor)
MAAEPVEDNCINFVAMKFIDNTLYFIENLESDYFGKLESKLSVIRNLNDQVLFIDQGNRPLFEDMTDSDCRDNAPRTIFIISMYKDSQPRGMAVTISVKCEKISTLSCENKIISFKEMNPPDNIKDTKSDIIFFQRSVPGHDNKMQFESSSYEGYFLACEKERDLFKLILKKEDELGDRSIMFTVQNED

SEQ ID NO: 152 - skipped

SEQ ID NO: 153 - protein, 157 aa, Homo sapiens; identical to SEQ ID NO: 149
  Amino acid sequence of IL-18 isoform 2 (Mature)

SEQ ID NO: 154 - skipped

SEQ ID NO: 155 - DNA, 531 bp, Artificial Sequence
  Synthetic: Codon optimized sequence
atgtacaggatgcaactcctgtcttgcattgcactaagtcttgcacttgtcacaaacagttactttggcaagcttgaatctaaattatcagtcataagaaatttgaatgaccaagttctcttcattgaccaaggaaatcggcctctatttgaagatatgactgattctgactgtagagataatgcaccccggaccatatttattataagtatgtataaagatagccagcctagaggtatggctgtaactatctctgtgaagtgtgagaagatttcaactctctcctgtgagaacaagattatttcctttaaggaaatgaatcctcctgataacatcaaggatacaaagagtgacatcatattctttcagagaagtgtcccaggacatgataataagatgcaatttgaatcttcatcatacgaaggatactttctagcttgtgagaaagagagagacctgtttaaactcattttgaagaaagaggatgaattgggcgatagatctataatgttcactgttcagaacgaagac

SEQ ID NO: 156 - DNA, 546 bp, Artificial Sequence
  Synthetic: Codon optimized sequence
atggaaatctgcagaggcctccgcagtcacctaatcactctcctcctcttcctgttccattcagagacgatctgctactttggcaagcttgaatctaaattatcagtcataagaaatttgaatgaccaagttctcttcattgaccaaggaaatcggcctctatttgaagatatgactgattctgactgtagagataatgcaccccggaccatatttattataagtatgtataaagatagccagcctagaggtatggctgtaactatctctgtgaagtgtgagaagatttcaactctctcctgtgagaacaagattatttcctttaaggaaatgaatcctcctgataacatcaaggatacaaagagtgacatcatattctttcagagaagtgtcccaggacatgataataagatgcaatttgaatcttcatcatacgaaggatactttctagcttgtgagaaagagagagacctgtttaaactcattttgaagaaagaggatgaattgggcgatagatctataatgttcactgttcagaacgaagac

SEQ ID NO: 157 - DNA, 546 bp, Artificial Sequence
  Synthetic: Codon optimized sequence
atggaaatctgcagaggcctccgcagtcacctaatcactctcctcctcttcctgttccattcagagacgatctgctactttggcaagcttgaatctaaattatcagtcataagaaatttgaatgaccaagttctcttcattgaccaaggaaatcggcctctatttgaagatatgactgattctgactgtagagataatgcaccccggaccatatttattataagtatgtataaagatagccagcctagaggtatggctgtaactatctctgtgaagtgtgagaaaatttcaactctctcctgtgagaacaaaattatttcctttaaggaaatgaatcctcctgataacatcaaggatacaaagagtgacatcatattctttcagagaagtgtcccaggacatgataataagatgcaatttgaatcttcatcatacgaaggatactttctagcttgtgagaaagagagagacctttttaaactcattttgaagaaagaggatgaattgggggatagatctataatgttcactgttcaaaacgaagac

SEQ ID NO: 158 - DNA, 531 bp, Artificial Sequence
  Synthetic: Codon optimized sequence
atggcctggaccgttctcctcctcggcctcctctctcactgcacaggctctgtgacctcctactttggcaagcttgaatctaaattatcagtcataagaaatttgaatgaccaagttctcttcattgaccaaggaaatcggcctctatttgaagatatgactgattctgactgtagagataatgcaccccggaccatatttattataagtatgtataaagatagccagcctagaggtatggctgtaactatctctgtgaagtgtgagaaaatttcaactctctcctgtgagaacaaaattatttcctttaaggaaatgaatcctcctgataacatcaaggatacaaagagtgacatcatattctttcagagaagtgtcccaggacatgataataagatgcaatttgaatcttcatcatacgaaggatactttctagcttgtgagaaagagagagacctttttaaactcattttgaagaaagaggatgaattgggggatagatctataatgttcactgttcaaaacgaagac

SEQ ID NO: 159 - DNA, 531 bp, Artificial Sequence
  Synthetic: Codon optimized sequence
atgtacaggatgcaactcctgtcttgcattgcactaagtcttgcacttgtcacaaacagttactttggcaagcttgaatctaaattatcagtcataagaaatttgaatgaccaagttctcttcattgaccaaggaaatcggcctctatttgaagatatgactgattctgactgtagagataatgcaccccggaccatatttattataagtatgtataaagatagccagcctagaggtatggctgtaactatctctgtgaagtgtgagaaaatttcaactctctcctgtgagaacaaaattatttcctttaaggaaatgaatcctcctgataacatcaaggatacaaagagtgacatcatattctttcagagaagtgtcccaggacatgataataagatgcaatttgaatcttcatcatacgaaggatactttctagcttgtgagaaagagagagacctttttaaactcattttgaagaaagaggatgaattgggggatagatctataatgttcactgttcaaaacgaagac

SEQ ID NO: 160 - DNA, 531 bp, Artificial Sequence
  Synthetic: Codon optimized sequence
atgtacaggatgcaactcctgtcttgcattgcactaagtcttgcacttgtcacaaacagttactttggcaagcttgaatctaaattatcagtcataagaaatttgaatgaccaagttctcttcattgaccaaggaaatcggcctctatttgaagatatgactgattctgactgtagagataatgcaccccggaccatatttattataagtatgtataaagatagccagcctagaggtatggctgtaactatctctgtgaagtgtgagaaaatttcaactctctcctgtgagaacaaaattatttcctttaaggaaatgaatcctcctgataacatcaaggatacaaaaagtgacatcatattctttcagagaagtgtcccaggacatgataataagatgcaatttgaatcttcatcatacgaaggatactttctagcttgtgaaaaagagagagacctttttaaactcattttgaaaaaagaggatgaattgggggatagatctataatgttcactgttcaaaacgaagac

SEQ ID NO: 161 - DNA, 579 bp, Homo sapiens; identical to SEQ ID NO: 148
  human IL-18 nucleotide sequence

SEQ ID NO: 162 - DNA, 531 bp, Artificial Sequence
  Synthetic: Codon optimized murine IL-18
atgtacagcatgcagctcgcatcctgtgtcacattgacacttgtgctccttgtcaacagcaactttggccgacttcactgtacaaccgcagtaatacggaatataaatgaccaagttctcttcgttgacaaaagacagcctgtgttcgaggatatgactgatattgatcaaagtgccagtgaaccccagaccagactgataatatacatgtacaaagacagtgaagtaagaggactggctgtgaccctctctgtgaaggatagtaaaatgtctaccctctcctgtaagaacaagatcatttcctttgaggaaatggatccacctgaaaatattgatgatatacaaagtgatctcatattctttcagaaacgtgttccaggacacaacaagatggagtttgaatcttcactgtatgaaggacactttcttgcttgccaaaaggaagatgatgctttcaaactcattctgaaaaaaaaggatgaaaatggggataaatctgtaatgttcactctcactaacttacatcaaagt

SEQ ID NO: 163 - protein, 25 aa, Artificial Sequence
  Synthetic: linker
  SITE 6..25: Repeats of "Glu Ala Ala Ala Lys" may or may not be present
EAAAKEAAAKEAAAKEAAAKEAAAK

SEQ ID NO: 164 - protein, 15 aa, Artificial Sequence
  Synthetic: linker
EAAAKEAAAKEAAAK

SEQ ID NO: 165 - protein, 5 aa, Artificial Sequence
  Synthetic: linker
GGGGG

SEQ ID NO: 166 - protein, 6 aa, Artificial Sequence
  Synthetic: linker
GGGGGG

SEQ ID NO: 167 - protein, 7 aa, Artificial Sequence
  Synthetic: linker
GGGGGGG

SEQ ID NO: 168 - protein, 8 aa, Artificial Sequence
  Synthetic: linker
GGGGGGGG

SEQ ID NO: 169 - protein, 16 aa, Artificial Sequence
  Synthetic: linker
GGGGSLVPRGSGGGGS

SEQ ID NO: 170 - protein, 6 aa, Artificial Sequence
  Synthetic: linker
GSGSGS

SEQ ID NO: 171 - protein, 15 aa, Artificial Sequence
  Synthetic: linker
GGGGSLVPRGSGGGG

SEQ ID NO: 172 - protein, 11 aa, Artificial Sequence
  Synthetic: linker
GGSGGHMGSGG

SEQ ID NO: 173 - protein, 11 aa, Artificial Sequence
  Synthetic: linker
GGSGGSGGSGG

SEQ ID NO: 174 - protein, 5 aa, Artificial Sequence
  Synthetic: linker
GGSGG

SEQ ID NO: 175 - protein, 8 aa, Artificial Sequence
  Synthetic: linker
GSGSGSGS

SEQ ID NO: 176 - protein, 18 aa, Artificial Sequence
  Synthetic: linker
GGGSEGGGSEGGGSEGGG

SEQ ID NO: 177 - protein, 8 aa, Artificial Sequence
  Synthetic: linker
AAGAATAA

SEQ ID NO: 178 - protein, 5 aa, Artificial Sequence
  Synthetic: linker
GGSSG

SEQ ID NO: 179 - protein, 11 aa, Artificial Sequence
  Synthetic: linker
GSGGGTGGGSG

SEQ ID NO: 180 - protein, 12 aa, Artificial Sequence
  Synthetic: linker
GSGSGSGSGGSG

SEQ ID NO: 181 - protein, 14 aa, Artificial Sequence
  Synthetic: linker
GSGGSGSGGSGGSG

SEQ ID NO: 182 - protein, 14 aa, Artificial Sequence
  Synthetic: linker
GSGGSGGSGGSGGS

SEQ ID NO: 183 - RNA, 1596 nt, Homo sapiens
  mRNA ORF for human IL-12
augugccaccagcagcuggugaucagcugguucagccugguguuccuggccagcccccugguggccaucugggagcugaagaaggacguguacgugguggaguuggauugguaccccgacgcccccggcgagaugguggugcugaccugcgacacccccgaggaggacggcaucaccuggacccuggaccagagcagcgaggugcugggcagcggcaagacccugaccauccaggugaaggaguucggcgacgccggccaguacaccugccacaagggcggcgaggugcugagccacagccugcugcugcugcacaagaaggaggacggcaucuggagcaccgacauccugaaggaccagaaggagcccaagaacaagaccuuccugagaugcgaggccaagaacuacagcggcagauucaccugcugguggcugaccaccaucagcaccgaccugaccuucagcgugaagagcagcagaggcagcagcgacccccagggcgugaccugcggcgccgccacccugagcgccgagagagugagaggcgacaacaaggaguacgaguacagcguggagugccaggaagauagcgccugccccgccgccgaggagagccugcccaucgaggugaugguggacgccgugcacaagcugaaguacgagaacuacaccagcagcuucuucaucagagauaucaucaagcccgacccccccaagaaccugcagcugaagccccugaagaacagccggcagguggaggugagcugggaguaccccgacaccuggagcaccccccacagcuacuucagccugaccuucugcgugcaggugcagggcaagagcaagagagagaagaaagauagaguguucaccgacaagaccagcgccaccgugaucugcagaaagaacgccagcaucagcgugagagcccaagauagauacuacagcagcagcuggagcgagugggccagcgugcccugcagcggcggcggcggcggcggcagcagaaaccugcccguggccacccccgaccccggcauguuccccugccugcaccacagccagaaccugcugagagccgugagcaacaugcugcagaaggcccggcagacccuggaguucuaccccugcaccagcgaggagaucgaccacgaagauaucaccaaagauaagaccagcaccguggaggccugccugccccuggagcugaccaagaacgagagcugccugaacagcagagagaccagcuucaucaccaacggcagcugccuggccagcagaaagaccagcuucaugauggcccugugccugagcagcaucuacgaggaccugaagauguaccagguggaguucaagaccaugaacgccaagcugcugauggaccccaagcggcagaucuuccuggaccagaacaugcuggccgugaucgacgagcugaugcaggcccugaacuucaacagcgagaccgugccccagaagagcagccuggaggagcccgacuucuacaagaccaagaucaagcugugcauccugcugcacgccuucagaaucagagccgugaccaucgacagagugaugagcuaccugaacgccagc

SEQ ID NO: 184 - protein, 306 aa, Artificial Sequence; identical to SEQ ID NO: 3
  Synthetic: Wildtype IL12B without signal amino acids

SEQ ID NO: 185 - DNA, 918 bp, Artificial Sequence
  Synthetic: Wildtype IL12B without signal nucleic acids
atatgggaactgaagaaagatgtttatgtcgtagaattggattggtatccggatgcccctggagaaatggtggtcctcacctgtgacacccctgaagaagatggtatcacctggaccttggaccagagcagtgaggtcttaggctctggcaaaaccctgaccatccaagtcaaagagtttggagatgctggccagtacacctgtcacaaaggaggcgaggttctaagccattcgctcctgctgcttcacaaaaaggaagatggaatttggtccactgatattttaaaggaccagaaagaacccaaaaataagacctttctaagatgcgaggccaagaattattctggacgtttcacctgctggtggctgacgacaatcagtactgatttgacattcagtgtcaaaagcagcagaggctcttctgacccccaaggggtgacgtgcggagctgctacactctctgcagagagagtcagaggggacaacaaggagtatgagtactcagtggagtgccaggaggacagtgcctgcccagctgctgaggagagtctgcccattgaggtcatggtggatgccgttcacaagctcaagtatgaaaactacaccagcagcttcttcatcagggacatcatcaaacctgacccacccaagaacttgcagctgaagccattaaagaattctcggcaggtggaggtcagctgggagtaccctgacacctggagtactccacattcctacttctccctgacattctgcgttcaggtccagggcaagagcaagagagaaaagaaagatagagtcttcacggacaagacctcagccacggtcatctgccgcaaaaatgccagcattagcgtgcgggcccaggaccgctactatagctcatcttggagcgaatgggcatctgtgccctgcagt

SEQ ID NO: 186 - protein, 197 aa, Artificial Sequence
  Synthetic: Wildtype IL12A without signal amino acids
RNLPVATPDPGMFPCLHHSQNLLRAVSNMLQKARQTLEFYPCTSEEIDHEDITKDKTSTVEACLPLELTKNESCLNSRETSFITNGSCLASRKTSFMMALCLSSIYEDLKMYQVEFKTMNAKLLMDPKRQIFLDQNMLAVIDELMQALNFNSETVPQKSSLEEPDFYKTKIKLCILLHAFRIRAVTIDRVMSYLNAS

SEQ ID NO: 187 - DNA, 591 bp, Artificial Sequence
  Synthetic: Wildtype IL12A without signal nucleic acids
agaaacctccccgtggccactccagacccaggaatgttcccatgccttcaccactcccaaaacctgctgagggccgtcagcaacatgctccagaaggccagacaaactctagaattttacccttgcacttctgaagagattgatcatgaagatatcacaaaagataaaaccagcacagtggaggcctgtttaccattggaattaaccaagaatgagagttgcctaaattccagagagacctctttcataactaatgggagttgcctggcctccagaaagacctcttttatgatggccctgtgccttagtagtatttatgaagacttgaagatgtaccaggtggagttcaagaccatgaatgcaaagcttctgatggatcctaagaggcagatctttctagatcaaaacatgctggcagttattgatgagctgatgcaggccctgaatttcaacagtgagactgtgccacaaaaatcctcccttgaagaaccggatttttataaaactaaaatcaagctctgcatacttcttcatgctttcagaattcgggcagtgactattgatagagtgatgagctatctgaatgcttcc

SEQ ID NO: 188 - protein, 22 aa, Artificial Sequence
  Synthetic: Wildtype IL12B signal peptide amino acids
MCHQQLVISWFSLVFLASPLVA

SEQ ID NO: 189 - DNA, 66 bp, Artificial Sequence
  Synthetic: Wildtype IL12B signal peptide nucleoic acids
atgtgtcaccagcagttggtcatctcttggttttccctggtttttctggcatctcccctcgtggcc

SEQ ID NO: 190 - protein, 10 aa, Artificial Sequence
  Synthetic: linker
GGSGGGGSGG

SEQ ID NO: 191 - protein, 8 aa, Artificial Sequence
  Synthetic: linker
GGSGGGGG

SEQ ID NO: 192 - protein, 8 aa, Artificial Sequence
  Synthetic: linker
GSGSGSGS

SEQ ID NO: 193 - protein, 2100 aa, Artificial Sequence
  SITE 1..2100: For every repeat of "GGGGGGGGGG GGGGGGGGGG S", at least one "G" is present and the others may be absent; the repeat of "GGGGGGGGGG GGGGGGGGGG S" is present at least once and may repeat up to 100 times or be absent
  Synthetic: linker
GGGGGGGGGGGGGGGGGGGGSGGGGGGGGGGGGGGGGGGGGSGGGGGGGGGGGGGGGGGGGGSGGGGGGGGGGGGGGGGGGGGSGGGGGGGGGGGGGGGGGGGGSGGGGGGGGGGGGGGGGGGGGSGGGGGGGGGGGGGGGGGGGGSGGGGGGGGGGGGGGGGGGGGSGGGGGGGGGGGGGGGGGGGGSGGGGGGGGGGGGGGGGGGGGSGGGGGGGGGGGGGGGGGGGGSGGGGGGGGGGGGGGGGGGGGSGGGGGGGGGGGGGGGGGGGGSGGGGGGGGGGGGGGGGGGGGSGGGGGGGGGGGGGGGGGGGGSGGGGGGGGGGGGGGGGGGGGSGGGGGGGGGGGGGGGGGGGGSGGGGGGGGGGGGGGGGGGGGSGGGGGGGGGGGGGGGGGGGGSGGGGGGGGGGGGGGGGGGGGSGGGGGGGGGGGGGGGGGGGGSGGGGGGGGGGGGGGGGGGGGSGGGGGGGGGGGGGGGGGGGGSGGGGGGGGGGGGGGGGGGGGSGGGGGGGGGGGGGGGGGGGGSGGGGGGGGGGGGGGGGGGGGSGGGGGGGGGGGGGGGGGGGGSGGGGGGGGGGGGGGGGGGGGSGGGGGGGGGGGGGGGGGGGGSGGGGGGGGGGGGGGGGGGGGSGGGGGGGGGGGGGGGGGGGGSGGGGGGGGGGGGGGGGGGGGSGGGGGGGGGGGGGGGGGGGGSGGGGGGGGGGGGGGGGGGGGSGGGGGGGGGGGGGGGGGGGGSGGGGGGGGGGGGGGGGGGGGSGGGGGGGGGGGGGGGGGGGGSGGGGGGGGGGGGGGGGGGGGSGGGGGGGGGGGGGGGGGGGGSGGGGGGGGGGGGGGGGGGGGSGGGGGGGGGGGGGGGGGGGGSGGGGGGGGGGGGGGGGGGGGSGGGGGGGGGGGGGGGGGGGGSGGGGGGGGGGGGGGGGGGGGSGGGGGGGGGGGGGGGGGGGGSGGGGGGGGGGGGGGGGGGGGSGGGGGGGGGGGGGGGGGGGGSGGGGGGGGGGGGGGGGGGGGSGGGGGGGGGGGGGGGGGGGGSGGGGGGGGGGGGGGGGGGGGSGGGGGGGGGGGGGGGGGGGGSGGGGGGGGGGGGGGGGGGGGSGGGGGGGGGGGGGGGGGGGGSGGGGGGGGGGGGGGGGGGGGSGGGGGGGGGGGGGGGGGGGGSGGGGGGGGGGGGGGGGGGGGSGGGGGGGGGGGGGGGGGGGGSGGGGGGGGGGGGGGGGGGGGSGGGGGGGGGGGGGGGGGGGGSGGGGGGGGGGGGGGGGGGGGSGGGGGGGGGGGGGGGGGGGGSGGGGGGGGGGGGGGGGGGGGSGGGGGGGGGGGGGGGGGGGGSGGGGGGGGGGGGGGGGGGGGSGGGGGGGGGGGGGGGGGGGGSGGGGGGGGGGGGGGGGGGGGSGGGGGGGGGGGGGGGGGGGGSGGGGGGGGGGGGGGGGGGGGSGGGGGGGGGGGGGGGGGGGGSGGGGGGGGGGGGGGGGGGGGSGGGGGGGGGGGGGGGGGGGGSGGGGGGGGGGGGGGGGGGGGSGGGGGGGGGGGGGGGGGGGGSGGGGGGGGGGGGGGGGGGGGSGGGGGGGGGGGGGGGGGGGGSGGGGGGGGGGGGGGGGGGGGSGGGGGGGGGGGGGGGGGGGGSGGGGGGGGGGGGGGGGGGGGSGGGGGGGGGGGGGGGGGGGGSGGGGGGGGGGGGGGGGGGGGSGGGGGGGGGGGGGGGGGGGGSGGGGGGGGGGGGGGGGGGGGSGGGGGGGGGGGGGGGGGGGGSGGGGGGGGGGGGGGGGGGGGSGGGGGGGGGGGGGGGGGGGGSGGGGGGGGGGGGGGGGGGGGSGGGGGGGGGGGGGGGGGGGGSGGGGGGGGGGGGGGGGGGGGSGGGGGGGGGGGGGGGGGGGGSGGGGGGGGGGGGGGGGGGGGSGGGGGGGGGGGGGGGGGGGGSGGGGGGGGGGGGGGGGGGGGSGGGGGGGGGGGGGGGGGGGGSGGGGGGGGGGGGGGGGGGGGSGGGGGGGGGGGGGGGGGGGGSGGGGGGGGGGGGGGGGGGGGSGGGGGGGGGGGGGGGGGGGGSGGGGGGGGGGGGGGGGGGGGSGGGGGGGGGGGGGGGGGGGGSGGGGGGGGGGGGGGGGGGGGS

SEQ ID NO: 194 - protein, 4 aa, Artificial Sequence
  Synthetic: linker
GGGS

SEQ ID NO: 195 - protein, 15 aa, Artificial Sequence
  Synthetic: linker
EAAAKEAAAKEAAAK

SEQ ID NO: 196 - protein, 40 aa, Artificial Sequence
  Synthetic: linker
  SITE 2..40: Gly may or may not be present
GGGGGGGGGGGGGGGGGGGGGGGGGGGGGGGGGGGGGGGG

SEQ ID NO: 197 - DNA, 20 bp, Artificial Sequence
  Synthetic: oligonucleotide
  misc_feature 2..5: /note="n is a, c, g, or t"
  misc_feature 7..7: /note="n is a, c, g, or t"
  misc_feature 10..10: /note="n is a, c, g, or t"
  misc_feature 14..14: /note="n is a, c, g, or t"
  misc_feature 16..17: /note="n is a, c, g, or t"
  misc_feature 19..19: /note="n is a, c, g, or t"
gnnnnwncrnctcncnnwnd

SEQ ID NO: 198 - DNA, 18 bp, Artificial Sequence
  Synthetic: oligonucleotide
attgggcacccgtaaggg